European Patent Specification EP 3 541 408 B1, published November 13, 2024. Title: COMPOSITIONS AND METHODS FOR THE TREATMENT OF ABERRANT ANGIOGENESIS. Applicant: The Schepens Eye Research Institute, Inc. The sequence listing filed with the application follows.

SEQUENCE LISTING (257 sequences)

SEQ ID NO: 1 - protein, 453 aa, Homo sapiens
MRIPVDASTSRRFTPPSTALSPGKMSEALPLGAPDAGAALAGKLRSGDRSMVEVLADHPGELVRTDSPNFLCSVLPTHWRCNKTLPIAFKVVALGDVPDGTLVTVMAGNDENYSAELRNATAAMKNQVARFNDLRFVGRSGRGKSFTLTITVFTNPPQVATYHRAIKITVDGPREPRRHRQKLDDQTKPGSLSFSERLSELEQLRRTAMRVSPHHPAPTPNPRASLNHSTAFNPQPQSQMQDTRQIQPSPPWSYDQSYQYLGSIASPSVHPATPISPGRASGMTTLSAELSSRLSTAPDLTAFSDPRQFPALPSISDPRMHYPGAFTYSPTPVTSGIGIGMSAMGSATRYHTYLPPPYPGSSQAQGGPFQASSPSYHLYYGASAGSYQFSMVGGERSPPRILPPCTNASTGSALLNPSLPNQSDVVEAEGSHSNSPTNMAPSARLEEAVWRPY

SEQ ID NO: 2 - protein, 472 aa, Homo sapiens
MRIPVDASTSRRFTPPSTALSPGKMSEALPLGAPDAGAALAGKLRSGDRSMVEVLADHPGELVRTDSPNFLCSVLPTHWRCNKTLPIAFKVVALGDVPDGTLVTVMAGNDENYSAELRNATAAMKNQVARFNDLRFVGRSGRGKSFTLTITVFTNPPQVATYHRAIKITVDGPREPRRHRQKLDDQTKPGSLSFSERLSELEQLRRTAMRVSPHHPAPTPNPRASLNHSTAFNPQPQSQMQDTRQIQPSPPWSYDQSYQYLGSIASPSVHPATPISPGRASGMTTLSAELSSRLSTAPDLTAFSDPRQFPALPSISDPRMHYPGAFTYSPTPVTSGIGIGMSAMGSATRYHTYLPPPYPGSSQAQGGPFQASSPSYHLYYGASAGSYQFSMVGGERSPPRILPPCTNASTGSALLNPSLPNQSDVVEAEGSHSNSPTNMGGASCSRQARRDPGPWARTPSWGRGRPTDRISL

SEQ ID NO: 3 - protein, 250 aa, Homo sapiens
MRIPVDASTSRRFTPPSTALSPGKMSEALPLGAPDAGAALAGKLRSGDRSMVEVLADHPGELVRTDSPNFLCSVLPTHWRCNKTLPIAFKVVALGDVPDGTLVTVMAGNDENYSAELRNATAAMKNQVARFNDLRFVGRSGRGKSFTLTITVFTNPPQVATYHRAIKITVDGPREPRRHRQKLDDQTKPGSLSFSERLSELEQLRRTAMRVSPHHPAPTPNPRASLNHSTAFNPQPQSQMQEEDTAPWRC

SEQ ID NO: 4 - protein, 257 aa, Homo sapiens
MRIPVDASTSRRFTPPSTALSPGKMSEALPLGAPDAGAALAGKLRSGDRSMVEVLADHPGELVRTDSPNFLCSVLPTHWRCNKTLPIAFKVVALGDVPDGTLVTVMAGNDENYSAELRNATAAMKNQVARFNDLRFVGRSGRGKSFTLTITVFTNPPQVATYHRAIKITVDGPREPRRHRQKLDDQTKPGSLSFSERLSELEQLRRTAMRVSPHHPAPTPNPRASLNHSTAFNPQPQSQMQDTRQIQPSPPWSYDQS

SEQ ID NO: 5 - protein, 224 aa, Homo sapiens
MRIPVDASTSRRFTPPSTALSPGKMSEALPLGAPDAGAALAGKLRSGDRSMVEVLADHPGELVRTDSPNFLCSVLPTHWRCNKTLPIAFKVVALGDVPDGTLVTVMAGNDENYSAELRNATAAMKNQVARFNDLRFVGRSGRGKSFTLTITVFTNPPQVATYHRAIKITVDGPREPRSKCIHLGLVHPPGWYTLQAGILRDHVSDSLGSTFPPGGWQAPVKPKS

SEQ ID NO: 6 - protein, 188 aa, Homo sapiens
MRIPVDASTSRRFTPPSTALSPGKMSEALPLGAPDAGAALAGKLRSGDRSMVEVLADHPGELVRTDSPNFLCSVLPTHWRCNKTLPIAFKVVALGDVPDGTLVTVMAGNDENYSAELRNATAAMKNQVARFNDLRFVGRSGRGKSFTLTITVFTNPPQVATYHRAIKITVDGPREPRNSLTWPRYPHI

SEQ ID NO: 7 - protein, 242 aa, Homo sapiens
MRIPVDASTSRRFTPPSTALSPGKMSEALPLGAPDAGAALAGKLRSGDRSMVEVLADHPGELVRTDSPNFLCSVLPTHWRCNKTLPIAFKVVALGDVPDGTLVTVMAGNDENYSAELRNATAAMKNQVARFNDLRFVDGPREPRRHRQKLDDQTKPGSLSFSERLSELEQLRRTAMRVSPHHPAPTPNPRASLNHSTAFNPQPQSQMQDTRQIQPSPPWSYDQSYQYLGSIASPSVHPATPI

SEQ ID NO: 8 - protein, 480 aa, Homo sapiens
MASDSIFESFPSYPQCFMRECILGMNPSRDVHDASTSRRFTPPSTALSPGKMSEALPLGAPDAGAALAGKLRSGDRSMVEVLADHPGELVRTDSPNFLCSVLPTHWRCNKTLPIAFKVVALGDVPDGTLVTVMAGNDENYSAELRNATAAMKNQVARFNDLRFVGRSGRGKSFTLTITVFTNPPQVATYHRAIKITVDGPREPRRHRQKLDDQTKPGSLSFSERLSELEQLRRTAMRVSPHHPAPTPNPRASLNHSTAFNPQPQSQMQDTRQIQPSPPWSYDQSYQYLGSIASPSVHPATPISPGRASGMTTLSAELSSRLSTAPDLTAFSDPRQFPALPSISDPRMHYPGAFTYSPTPVTSGIGIGMSAMGSATRYHTYLPPPYPGSSQAQGGPFQASSPSYHLYYGASAGSYQFSMVGGERSPPRILPPCTNASTGSALLNPSLPNQSDVVEAEGSHSNSPTNMAPSARLEEAVWRPY

SEQ ID NO: 9 - protein, 456 aa, Homo sapiens
MNPSRDVHDASTSRRFTPPSTALSPGKMSEALPLGAPDAGAALAGKLRSGDRSMVEVLADHPGELVRTDSPNFLCSVLPTHWRCNKTLPIAFKVVALGDVPDGTLVTVMAGNDENYSAELRNATAAMKNQVARFNDLRFVGRSGRGKSFTLTITVFTNPPQVATYHRAIKITVDGPREPRRHRQKLDDQTKPGSLSFSERLSELEQLRRTAMRVSPHHPAPTPNPRASLNHSTAFNPQPQSQMQDTRQIQPSPPWSYDQSYQYLGSIASPSVHPATPISPGRASGMTTLSAELSSRLSTAPDLTAFSDPRQFPALPSISDPRMHYPGAFTYSPTPVTSGIGIGMSAMGSATRYHTYLPPPYPGSSQAQGGPFQASSPSYHLYYGASAGSYQFSMVGGERSPPRILPPCTNASTGSALLNPSLPNQSDVVEAEGSHSNSPTNMAPSARLEEAVWRPY

SEQ ID NO: 10 - protein, 468 aa, Homo sapiens
MPAAPRGPAQGEAAARTRSRDASTSRRFTPPSTALSPGKMSEALPLGAPDAGAALAGKLRSGDRSMVEVLADHPGELVRTDSPNFLCSVLPTHWRCNKTLPIAFKVVALGDVPDGTLVTVMAGNDENYSAELRNATAAMKNQVARFNDLRFVGRSGRGKSFTLTITVFTNPPQVATYHRAIKITVDGPREPRRHRQKLDDQTKPGSLSFSERLSELEQLRRTAMRVSPHHPAPTPNPRASLNHSTAFNPQPQSQMQDTRQIQPSPPWSYDQSYQYLGSIASPSVHPATPISPGRASGMTTLSAELSSRLSTAPDLTAFSDPRQFPALPSISDPRMHYPGAFTYSPTPVTSGIGIGMSAMGSATRYHTYLPPPYPGSSQAQGGPFQASSPSYHLYYGASAGSYQFSMVGGERSPPRILPPCTNASTGSALLNPSLPNQSDVVEAEGSHSNSPTNMAPSARLEEAVWRPY

SEQ ID NO: 11 - protein, 348 aa, Homo sapiens
MAGNDENYSAELRNATAAMKNQVARFNDLRFVGRSGRGKSFTLTITVFTNPPQVATYHRAIKITVDGPREPRRHRQKLDDQTKPGSLSFSERLSELEQLRRTAMRVSPHHPAPTPNPRASLNHSTAFNPQPQSQMQDTRQIQPSPPWSYDQSYQYLGSIASPSVHPATPISPGRASGMTTLSAELSSRLSTAPDLTAFSDPRQFPALPSISDPRMHYPGAFTYSPTPVTSGIGIGMSAMGSATRYHTYLPPPYPGSSQAQGGPFQASSPSYHLYYGASAGSYQFSMVGGERSPPRILPPCTNASTGSALLNPSLPNQSDVVEAEGSHSNSPTNMAPSARLEEAVWRPY

SEQ ID NO: 12 - DNA, 7274 bp, Artificial Sequence
  RUNX1 cDNA Sequence
catagagccagcgggcgcgggcgggacgggcgccccgcggccggacccagccagggcaccacgctgcccggccctgcgccgccaggcacttctttccggggctcctagggacgccagaaggaagtcaacctctgctgcttctccttggcctgcgttggaccttcctttttttgttgtttttttttgtttttcccctttcttccttttgaattaactggcttcttggctggatgttttcaacttctttcctggctgcgaacttttccccaattgttttccttttacaacagggggagaaagtgctctgtggtccgaggcgagccgtgaagttgcgtgtgcgtggcagtgtgcgtggcaggatgtgcgtgcgtgtgtaacccgagccgcccgatctgtttcgatctgcgccgcggagccctccctcaaggcccgctccacctgctgcggttacgcggcgctcgtgggtgttcgtgcctcggagcagctaaccggcgggtgctgggcgacggtggaggagtatcgtctcgctgctgcccgagtcagggctgagtcacccagctgatgtagacagtggctgccttccgaagagtgcgtgtttgcatgtgtgtgactctgcggctgctcaactcccaacaaaccagaggaccagccacaaacttaaccaacatccccaaacccgagttcacagatgtgggagagctgtagaaccctgagtgtcatcgactgggccttcttatgattgttgttttaagattagctgaagatctctgaaacgctgaattttctgcactgagcgttttgacagaattcattgagagaacagagaacatgacaagtacttctagctcagcactgctccaactactgaagctgattttcaaggctacttaaaaaaatctgcagcgtacattaatggatttctgttgtgtttaaattctccacagattgtattgtaaatattttatgaagtagagcatatgtatatatttatatatacgtgcacatacattagtagcactacctttggaagtctcagctcttgcttttcgggactgaagccagttttgcatgataaaagtggccttgttacgggagataattgtgttctgttgggactttagacaaaactcacctgcaaaaaactgacaggcattaactactggaacttccaaataatgtgtttgctgatcgttttactcttcgcataaatattttaggaagtgtatgagaattttgccttcaggaacttttctaacagccaaagacagaacttaacctctgcaagcaagattcgtggaagatagtctccactttttaatgcactaagcaatcggttgctaggagcccatcctgggtcagaggccgatccgcagaaccagaacgttttcccctcctggactgttagtaacttagtctccctcctcccctaaccacccccgcccccccccaccccccgcagtaataaaggcccctgaacgtgtatgttggtctcccgggagctgcttgctgaagatccgcgcccctgtcgccgtctggtaggagctgtttgcagggtcctaactcaatcggcttgttgtgatgcgtatccccgtagatgccagcacgagccgccgcttcacgccgccttccaccgcgctgagcccaggcaagatgagcgaggcgttgccgctgggcgccccggacgccggcgctgccctggccggcaagctgaggagcggcgaccgcagcatggtggaggtgctggccgaccacccgggcgagctggtgcgcaccgacagccccaacttcctctgctccgtgctgcctacgcactggcgctgcaacaagaccctgcccatcgctttcaaggtggtggccctaggggatgttccagatggcactctggtcactgtgatggctggcaatgatgaaaactactcggctgagctgagaaatgctaccgcagccatgaagaaccaggttgcaagatttaatgacctcaggtttgtcggtcgaagtggaagagggaaaagcttcactctgaccatcactgtcttcacaaacccaccgcaagtcgccacctaccacagagccatcaaaatcacagtggatgggccccgagaacctcgaagacatcggcagaaactagatgatcagaccaagcccgggagcttgtccttttccgagcggctcagtgaactggagcagctgcggcgcacagccatgagggtcagcccacaccacccagcccccacgcccaaccctcgtgcctccctgaaccactccactgcctttaaccctcagcctcagagtcagatgcaggatacaaggcagatccaaccatccccaccgtggtcctacgatcagtcctaccaatacctgggatccattgcctctccttctgtgcacccagcaacgcccatttcacctggacgtgccagcggcatgacaaccctctctgcagaactttccagtcgactctcaacggcacccgacctgacagcgttcagcgacccgcgccagttccccgcgctgccctccatctccgacccccgcatgcactatccaggcgccttcacctactccccgacgccggtcacctcgggcatcggcatcggcatgtcggccatgggctcggccacgcgctaccacacctacctgccgccgccctaccccggctcgtcgcaagcgcagggaggcccgttccaagccagctcgccctcctaccacctgtactacggcgcctcggccggctcctaccagttctccatggtgggcggcgagcgctcgccgccgcgcatcctgccgccctgcaccaacgcctccaccggctccgcgctgctcaaccccagcctcccgaaccagagcgacgtggtggaggccgagggcagccacagcaactcccccaccaacatggcgccctccgcgcgcctggaggaggccgtgtggaggccctactgaggcgccaggcctggcccggctgggccccgcgggccgccgccttcgcctccgggcgcgcgggcctcctgttcgcgacaagcccgccgggatcccgggccctgggcccggccaccgtcctggggccgagggcgcccgacggccaggatctcgctgtaggtcaggcccgcgcagcctcctgcgcccagaagcccacgccgccgccgtctgctggcgccccggccctcgcggaggtgtccgaggcgacgcacctcgagggtgtccgccggccccagcacccaggggacgcgctggaaagcaaacaggaagattcccggagggaaactgtgaatgcttctgatttagcaatgctgtgaataaaaagaaagattttatacccttgacttaactttttaaccaagttgtttattccaaagagtgtggaattttggttggggtggggggagaggagggatgcaactcgccctgtttggcatctaattcttatttttaatttttccgcaccttatcaattgcaaaatgcgtatttgcatttgggtggtttttatttttatatacgtttatataaatatatataaattgagcttgcttctttcttgctttgaccatggaaagaaatatgattcccttttctttaagttttatttaacttttcttttggacttttgggtagttgtttttttttgttttgttttgtttttttgagaaacagctacagctttgggtcatttttaactactgtattcccacaaggaatccccagatatttatgtatcttgatgttcagacatttatgtgttgataattttttaattatttaaatgtacttatattaagaaaaatatcaagtactacattttcttttgttcttgatagtagccaaagttaaatgtatcacattgaagaaggctagaaaaaaagaatgagtaatgtgatcgcttggttatccagaagtattgtttacattaaactccctttcatgttaatcaaacaagtgagtagctcacgcagcaacgtttttaataggatttttagacactgagggtcactccaaggatcagaagtatggaattttctgccaggctcaacaagggtctcatatctaacttcctccttaaaacagagaaggtcaatctagttccagagggttgaggcaggtgccaataattacatctttggagaggatttgatttctgcccagggatttgctcaccccaaggtcatctgataatttcacagatgctgtgtaacagaacacagccaaagtaaactgtgtaggggagccacatttacataggaaccaaatcaatgaatttaggggttacgattatagcaatttaagggcccaccagaagcaggcctcgaggagtcaatttgcctctgtgtgcctcagtggagacaagtgggaaaacatggtcccacctgtgcgagaccccctgtcctgtgctgctcactcaacaacatctttgtgttgctttcaccaggctgagaccctaccctatggggtatatgggcttttacctgtgcaccagtgtgacaggaaagattcatgtcactactgtccgtggctacaattcaaaggtatccaatgtcgctgtaaattttatggcactatttttattggaggatttggtcagaatgcagttgttgtacaactcataaatactaactgctgattttgacacatgtgtgctccaaatgatctggtggttatttaacgtacctcttaaaattcgttgaaacgatttcaggtcaactctgaagagtatttgaaagcaggacttcagaacagtgtttgatttttattttataaatttaagcattcaaattaggcaaatctttggctgcaggcagcaaaaacagctggacttatttaaaacaacttgtttttgagttttcttatatatatattgattatttgttttacacacatgcagtagcactttggtaagagttaaagagtaaagcagcttatgttgtcaggtcgttcttatctagagaagagctatagcagatctcggacaaactcagaatatattcactttcatttttgacaggattccctccacaactcagtttcatatattattccgtattacatttttgcagctaaattaccataaaatgtcagcaaatgtaaaaatttaatttctgaaaagcaccattagcccatttcccccaaattaaacgtaaatgttttttttcagcacatgttaccatgtctgacctgcaaaaatgctggagaaaaatgaaggaaaaaattatgtttttcagtttaattctgttaactgaagatattccaactcaaaaccagcctcatgctctgattagataatcttttacattgaacctttactctcaaagccatgtgtggagggggcttgtcactattgtaggctcactggattggtcatttagagtttcacagactcttaccagcatatatagtatttaattgtttcaaaaaaaatcaaactgtagttgttttggcgataggtctcacgcaacacatttttgtatgtgtgtgtgtgtgcgtgtgtgtgtgtgtgtgtgaaaaattgcattcattgacttcaggtagattaaggtatctttttattcattgccctcaggaaagttaaggtatcaatgagacccttaagccaatcatgtaataactgcatgtgtctggtccaggagaagtattgaataagccatttctactgcttactcatgtccctatttatgatttcaacatggatacatatttcagttctttctttttctcactatctgaaaatacatttccctccctctcttccccccaatatctccctttttttctctcttcctctatcttccaaaccccactttctccctcctccttttcctgtgttctcttaagcagatagcacatacccccacccagtaccaaatttcagaacacaagaaggtccagttcttcccccttcacataaaggaacatggtttgtcagcctttctcctgtttatgggtttcttccagcagaacagagacattgccaaccatattggatctgcttgctgtccaaaccagcaaactttcctgggcaaatcacaatcagtgagtaaatagacagcctttctgctgccttgggtttctgtgcagataaacagaaatgctctgattagaaaggaaatgaatggttccactcaaatgtcctgcaatttaggattgcagatttctgccttgaaatacctgtttctttgggacattccgtcctgatgatttttatttttgttggtttttatttttggggggaatgacatgtttgggtcttttatacatgaaaatttgtttgacaataatctcacaaaacatattttacatctgaacaaaatgcctttttgtttaccgtagcgtatacatttgttttgggatttttgtgtgtttgttgggaattttgtttttagccaggtcagtattgatgaggctgatcatttggctctttttttccttccagaagagttgcatcaacaaagttaattgtatttatgtatgtaaatagattttaagcttcattataaaatattgttaatgcctataactttttttcaatttttttgtgtgtgtttctaaggactttttcttaggtttgctaaatactgtagggaaaaaaatgcttctttctactttgtttattttagactttaaaatgagctacttcttattcacttttgtaaacagctaatagcatggttccaattttttttaagttcactttttttgttctaggggaaatgaatgtgcaaaaaaagaaaaagaactgttggttatttgtgttattctggatgtataaaaatcaatggaaaaaaataaactttcaaattgaaatgacggtataacacatctactgaaaaagcaacgggaaatgtggtcctatttaagccagcccccacctagggtctatttgtgtggcagttattgggtttggtcacaaaacatcctgaaaattcgtgcgtgggcttctttctccctggtacaaacgtatggaatgcttcttaaaggggaactgtcaagctggtgtcttcagccagatgacatgagagaatatcccagaaccctctctccaaggtgtttctagatagcacaggagagcaggcactgcactgtccacagtccacggtacacagtcgggtgggccgcctcccctctcctgggagcattcgtcgtgcccagcctgagcagggcagctggactgctgctgttcaggagccaccagagccttcctctctttgtaccacagtttcttctgtaaatccagtgttacaatcagtgtgaatggcaaataaacagtttgacaagtacatacaccata

SEQ ID NO: 13 - DNA, 5967 bp, Artificial Sequence
  RUNX1 cDNA sequence
ctttgggcctcataaacaaccacagaaccacaagttgggtagcctggcagtgtcagaagtctgaacccagcatagtggtcagcaggcaggacgaatcacactgaatgcaaaccacagggtttcgcagcgtggtaaaagaaatcattgagtcccccgccttcagaagagggtgcattttcaggaggaagcgatggcttcagacagcatatttgagtcatttccttcgtacccacagtgcttcatgagagaatgcatacttggaatgaatccttctagagacgtccacgatgccagcacgagccgccgcttcacgccgccttccaccgcgctgagcccaggcaagatgagcgaggcgttgccgctgggcgccccggacgccggcgctgccctggccggcaagctgaggagcggcgaccgcagcatggtggaggtgctggccgaccacccgggcgagctggtgcgcaccgacagccccaacttcctctgctccgtgctgcctacgcactggcgctgcaacaagaccctgcccatcgctttcaaggtggtggccctaggggatgttccagatggcactctggtcactgtgatggctggcaatgatgaaaactactcggctgagctgagaaatgctaccgcagccatgaagaaccaggttgcaagatttaatgacctcaggtttgtcggtcgaagtggaagagggaaaagcttcactctgaccatcactgtcttcacaaacccaccgcaagtcgccacctaccacagagccatcaaaatcacagtggatgggccccgagaacctcgaagacatcggcagaaactagatgatcagaccaagcccgggagcttgtccttttccgagcggctcagtgaactggagcagctgcggcgcacagccatgagggtcagcccacaccacccagcccccacgcccaaccctcgtgcctccctgaaccactccactgcctttaaccctcagcctcagagtcagatgcaggatacaaggcagatccaaccatccccaccgtggtcctacgatcagtcctaccaatacctgggatccattgcctctccttctgtgcacccagcaacgcccatttcacctggacgtgccagcggcatgacaaccctctctgcagaactttccagtcgactctcaacggcacccgacctgacagcgttcagcgacccgcgccagttccccgcgctgccctccatctccgacccccgcatgcactatccaggcgccttcacctactccccgacgccggtcacctcgggcatcggcatcggcatgtcggccatgggctcggccacgcgctaccacacctacctgccgccgccctaccccggctcgtcgcaagcgcagggaggcccgttccaagccagctcgccctcctaccacctgtactacggcgcctcggccggctcctaccagttctccatggtgggcggcgagcgctcgccgccgcgcatcctgccgccctgcaccaacgcctccaccggctccgcgctgctcaaccccagcctcccgaaccagagcgacgtggtggaggccgagggcagccacagcaactcccccaccaacatggcgccctccgcgcgcctggaggaggccgtgtggaggccctactgaggcgccaggcctggcccggctgggccccgcgggccgccgccttcgcctccgggcgcgcgggcctcctgttcgcgacaagcccgccgggatcccgggccctgggcccggccaccgtcctggggccgagggcgcccgacggccaggatctcgctgtaggtcaggcccgcgcagcctcctgcgcccagaagcccacgccgccgccgtctgctggcgccccggccctcgcggaggtgtccgaggcgacgcacctcgagggtgtccgccggccccagcacccaggggacgcgctggaaagcaaacaggaagattcccggagggaaactgtgaatgcttctgatttagcaatgctgtgaataaaaagaaagattttatacccttgacttaactttttaaccaagttgtttattccaaagagtgtggaattttggttggggtggggggagaggagggatgcaactcgccctgtttggcatctaattcttatttttaatttttccgcaccttatcaattgcaaaatgcgtatttgcatttgggtggtttttatttttatatacgtttatataaatatatataaattgagcttgcttctttcttgctttgaccatggaaagaaatatgattcccttttctttaagttttatttaacttttcttttggacttttgggtagttgtttttttttgttttgttttgtttttttgagaaacagctacagctttgggtcatttttaactactgtattcccacaaggaatccccagatatttatgtatcttgatgttcagacatttatgtgttgataattttttaattatttaaatgtacttatattaagaaaaatatcaagtactacattttcttttgttcttgatagtagccaaagttaaatgtatcacattgaagaaggctagaaaaaaagaatgagtaatgtgatcgcttggttatccagaagtattgtttacattaaactccctttcatgttaatcaaacaagtgagtagctcacgcagcaacgtttttaataggatttttagacactgagggtcactccaaggatcagaagtatggaattttctgccaggctcaacaagggtctcatatctaacttcctccttaaaacagagaaggtcaatctagttccagagggttgaggcaggtgccaataattacatctttggagaggatttgatttctgcccagggatttgctcaccccaaggtcatctgataatttcacagatgctgtgtaacagaacacagccaaagtaaactgtgtaggggagccacatttacataggaaccaaatcaatgaatttaggggttacgattatagcaatttaagggcccaccagaagcaggcctcgaggagtcaatttgcctctgtgtgcctcagtggagacaagtgggaaaacatggtcccacctgtgcgagaccccctgtcctgtgctgctcactcaacaacatctttgtgttgctttcaccaggctgagaccctaccctatggggtatatgggcttttacctgtgcaccagtgtgacaggaaagattcatgtcactactgtccgtggctacaattcaaaggtatccaatgtcgctgtaaattttatggcactatttttattggaggatttggtcagaatgcagttgttgtacaactcataaatactaactgctgattttgacacatgtgtgctccaaatgatctggtggttatttaacgtacctcttaaaattcgttgaaacgatttcaggtcaactctgaagagtatttgaaagcaggacttcagaacagtgtttgatttttattttataaatttaagcattcaaattaggcaaatctttggctgcaggcagcaaaaacagctggacttatttaaaacaacttgtttttgagttttcttatatatatattgattatttgttttacacacatgcagtagcactttggtaagagttaaagagtaaagcagcttatgttgtcaggtcgttcttatctagagaagagctatagcagatctcggacaaactcagaatatattcactttcatttttgacaggattccctccacaactcagtttcatatattattccgtattacatttttgcagctaaattaccataaaatgtcagcaaatgtaaaaatttaatttctgaaaagcaccattagcccatttcccccaaattaaacgtaaatgttttttttcagcacatgttaccatgtctgacctgcaaaaatgctggagaaaaatgaaggaaaaaattatgtttttcagtttaattctgttaactgaagatattccaactcaaaaccagcctcatgctctgattagataatcttttacattgaacctttactctcaaagccatgtgtggagggggcttgtcactattgtaggctcactggattggtcatttagagtttcacagactcttaccagcatatatagtatttaattgtttcaaaaaaaatcaaactgtagttgttttggcgataggtctcacgcaacacatttttgtatgtgtgtgtgtgtgcgtgtgtgtgtgtgtgtgtgaaaaattgcattcattgacttcaggtagattaaggtatctttttattcattgccctcaggaaagttaaggtatcaatgagacccttaagccaatcatgtaataactgcatgtgtctggtccaggagaagtattgaataagccatttctactgcttactcatgtccctatttatgatttcaacatggatacatatttcagttctttctttttctcactatctgaaaatacatttccctccctctcttccccccaatatctccctttttttctctcttcctctatcttccaaaccccactttctccctcctccttttcctgtgttctcttaagcagatagcacatacccccacccagtaccaaatttcagaacacaagaaggtccagttcttcccccttcacataaaggaacatggtttgtcagcctttctcctgtttatgggtttcttccagcagaacagagacattgccaaccatattggatctgcttgctgtccaaaccagcaaactttcctgggcaaatcacaatcagtgagtaaatagacagcctttctgctgccttgggtttctgtgcagataaacagaaatgctctgattagaaaggaaatgaatggttccactcaaatgtcctgcaatttaggattgcagatttctgccttgaaatacctgtttctttgggacattccgtcctgatgatttttatttttgttggtttttatttttggggggaatgacatgtttgggtcttttatacatgaaaatttgtttgacaataatctcacaaaacatattttacatctgaacaaaatgcctttttgtttaccgtagcgtatacatttgttttgggatttttgtgtgtttgttgggaattttgtttttagccaggtcagtattgatgaggctgatcatttggctctttttttccttccagaagagttgcatcaacaaagttaattgtatttatgtatgtaaatagattttaagcttcattataaaatattgttaatgcctataactttttttcaatttttttgtgtgtgtttctaaggactttttcttaggtttgctaaatactgtagggaaaaaaatgcttctttctactttgtttattttagactttaaaatgagctacttcttattcacttttgtaaacagctaatagcatggttccaattttttttaagttcactttttttgttctaggggaaatgaatgtgcaaaaaaagaaaaagaactgttggttatttgtgttattctggatgtataaaaatcaatggaaaaaaataaactttcaaattgaaatgacggtataacacatctactgaaaaagcaacgggaaatgtggtcctatttaagccagcccccacctagggtctatttgtgtggcagttattgggtttggtcacaaaacatcctgaaaattcgtgcgtgggcttctttctccctggtacaaacgtatggaatgcttcttaaaggggaactgtcaagctggtgtcttcagccagatgacatgagagaatatcccagaaccctctctccaaggtgtttctagatagcacaggagagcaggcactgcactgtccacagtccacggtacacagtcgggtgggccgcctcccctctcctgggagcattcgtcgtgcccagcctgagcagggcagctggactgctgctgttcaggagccaccagagccttcctctctttgtaccacagtttcttctgtaaatccagtgttacaatcagtgtgaatggcaaataaacagtttgacaagtacatacaccata

SEQ ID NO: 14 - DNA, 2722 bp, Artificial Sequence
  RUNX1 cDNA sequence
catagagccagcgggcgcgggcgggacgggcgccccgcggccggacccagccagggcaccacgctgcccggccctgcgccgccaggcacttctttccggggctcctagggacgccagaaggaagtcaacctctgctgcttctccttggcctgcgttggaccttcctttttttgttgtttttttttgtttttcccctttcttccttttgaattaactggcttcttggctggatgttttcaacttctttcctggctgcgaacttttccccaattgttttccttttacaacagggggagaaagtgctctgtggtccgaggcgagccgtgaagttgcgtgtgcgtggcagtgtgcgtggcaggatgtgcgtgcgtgtgtaacccgagccgcccgatctgtttcgatctgcgccgcggagccctccctcaaggcccgctccacctgctgcggttacgcggcgctcgtgggtgttcgtgcctcggagcagctaaccggcgggtgctgggcgacggtggaggagtatcgtctcgctgctgcccgagtcagggctgagtcacccagctgatgtagacagtggctgccttccgaagagtgcgtgtttgcatgtgtgtgactctgcggctgctcaactcccaacaaaccagaggaccagccacaaacttaaccaacatccccaaacccgagttcacagatgtgggagagctgtagaaccctgagtgtcatcgactgggccttcttatgattgttgttttaagattagctgaagatctctgaaacgctgaattttctgcactgagcgttttgacagaattcattgagagaacagagaacatgacaagtacttctagctcagcactgctccaactactgaagctgattttcaaggctacttaaaaaaatctgcagcgtacattaatggatttctgttgtgtttaaattctccacagattgtattgtaaatattttatgaagtagagcatatgtatatatttatatatacgtgcacatacattagtagcactacctttggaagtctcagctcttgcttttcgggactgaagccagttttgcatgataaaagtggccttgttacgggagataattgtgttctgttgggactttagacaaaactcacctgcaaaaaactgacaggcattaactactggaacttccaaataatgtgtttgctgatcgttttactcttcgcataaatattttaggaagtgtatgagaattttgccttcaggaacttttctaacagccaaagacagaacttaacctctgcaagcaagattcgtggaagatagtctccactttttaatgcactaagcaatcggttgctaggagcccatcctgggtcagaggccgatccgcagaaccagaacgttttcccctcctggactgttagtaacttagtctccctcctcccctaaccacccccgcccccccccaccccccgcagtaataaaggcccctgaacgtgtatgttggtctcccgggagctgcttgctgaagatccgcgcccctgtcgccgtctggtaggagctgtttgcagggtcctaactcaatcggcttgttgtgatgcgtatccccgtagatgccagcacgagccgccgcttcacgccgccttccaccgcgctgagcccaggcaagatgagcgaggcgttgccgctgggcgccccggacgccggcgctgccctggccggcaagctgaggagcggcgaccgcagcatggtggaggtgctggccgaccacccgggcgagctggtgcgcaccgacagccccaacttcctctgctccgtgctgcctacgcactggcgctgcaacaagaccctgcccatcgctttcaaggtggtggccctaggggatgttccagatggcactctggtcactgtgatggctggcaatgatgaaaactactcggctgagctgagaaatgctaccgcagccatgaagaaccaggttgcaagatttaatgacctcaggtttgtcggtcgaagtggaagagggaaaagcttcactctgaccatcactgtcttcacaaacccaccgcaagtcgccacctaccacagagccatcaaaatcacagtggatgggccccgagaacctcgaagacatcggcagaaactagatgatcagaccaagcccgggagcttgtccttttccgagcggctcagtgaactggagcagctgcggcgcacagccatgagggtcagcccacaccacccagcccccacgcccaaccctcgtgcctccctgaaccactccactgcctttaaccctcagcctcagagtcagatgcaggaggaagacacagcaccctggagatgttaaggcagaagtcagttcttctgtccatccctctccccagccaggatagagctatcttttccatctcatcctcagaagagactcagaagaaagatgacagccctcagaatgcacgttatgaggaaggcagaatgtgggtctgtaattcctccgtgtcccttctccccctctgcaaaccgtcgtaacaataatagttcctaacacatgggacaattgtgaggattaaatgagttagcctgcagaaatcacttgatgcacagcacatgggaagcattgtgtgtatttattaatccttcacaaagtctttgagatatatttttatcaaatatttagcatggatcccggtacactttcaatacttaataaatggtcaatgttattctttttcactatt

SEQ ID NO: 15 - DNA, 6230 bp, Artificial Sequence
  RUNX1 cDNA sequence
agggcggctgctgccccctggcgtccgccagagcccgcggcgcgtcccgacagctccgcgcagtccgggcccgcccgggaaaggcctccacgccagtcaaccccggccccctcctgcgtccgggcccgcggcaacgcccggggacagtccctgcgcggcagcggccacagcaccctagccctgggggagggaggagcgggcgtcaggggccccgtgaggtcggcgagggacccccgcgccggggagcttaattgaggggctccgcggggaccacaaagcagcccgcggtggaacggggccgggatccggggactgggttgcagccccggggtggatgagaggccccgggaggtgcagggcccggcagggagggcgtggagggactcatggtgacgggagcagcctccgctgggagggagccccgccgggcggggtcggagttggcagcgcacgccggaccgggggcggggccctccgagctccgcgaaaatgcccgcagcaccgcggggaccggcgcagggggaagcggccgcccgcacgcgaagccgggatgccagcacgagccgccgcttcacgccgccttccaccgcgctgagcccaggcaagatgagcgaggcgttgccgctgggcgccccggacgccggcgctgccctggccggcaagctgaggagcggcgaccgcagcatggtggaggtgctggccgaccacccgggcgagctggtgcgcaccgacagccccaacttcctctgctccgtgctgcctacgcactggcgctgcaacaagaccctgcccatcgctttcaaggtggtggccctaggggatgttccagatggcactctggtcactgtgatggctggcaatgatgaaaactactcggctgagctgagaaatgctaccgcagccatgaagaaccaggttgcaagatttaatgacctcaggtttgtcggtcgaagtggaagagggaaaagcttcactctgaccatcactgtcttcacaaacccaccgcaagtcgccacctaccacagagccatcaaaatcacagtggatgggccccgagaacctcgaagacatcggcagaaactagatgatcagaccaagcccgggagcttgtccttttccgagcggctcagtgaactggagcagctgcggcgcacagccatgagggtcagcccacaccacccagcccccacgcccaaccctcgtgcctccctgaaccactccactgcctttaaccctcagcctcagagtcagatgcaggatacaaggcagatccaaccatccccaccgtggtcctacgatcagtcctaccaatacctgggatccattgcctctccttctgtgcacccagcaacgcccatttcacctggacgtgccagcggcatgacaaccctctctgcagaactttccagtcgactctcaacggcacccgacctgacagcgttcagcgacccgcgccagttccccgcgctgccctccatctccgacccccgcatgcactatccaggcgccttcacctactccccgacgccggtcacctcgggcatcggcatcggcatgtcggccatgggctcggccacgcgctaccacacctacctgccgccgccctaccccggctcgtcgcaagcgcagggaggcccgttccaagccagctcgccctcctaccacctgtactacggcgcctcggccggctcctaccagttctccatggtgggcggcgagcgctcgccgccgcgcatcctgccgccctgcaccaacgcctccaccggctccgcgctgctcaaccccagcctcccgaaccagagcgacgtggtggaggccgagggcagccacagcaactcccccaccaacatggcgccctccgcgcgcctggaggaggccgtgtggaggccctactgaggcgccaggcctggcccggctgggccccgcgggccgccgccttcgcctccgggcgcgcgggcctcctgttcgcgacaagcccgccgggatcccgggccctgggcccggccaccgtcctggggccgagggcgcccgacggccaggatctcgctgtaggtcaggcccgcgcagcctcctgcgcccagaagcccacgccgccgccgtctgctggcgccccggccctcgcggaggtgtccgaggcgacgcacctcgagggtgtccgccggccccagcacccaggggacgcgctggaaagcaaacaggaagattcccggagggaaactgtgaatgcttctgatttagcaatgctgtgaataaaaagaaagattttatacccttgacttaactttttaaccaagttgtttattccaaagagtgtggaattttggttggggtggggggagaggagggatgcaactcgccctgtttggcatctaattcttatttttaatttttccgcaccttatcaattgcaaaatgcgtatttgcatttgggtggtttttatttttatatacgtttatataaatatatataaattgagcttgcttctttcttgctttgaccatggaaagaaatatgattcccttttctttaagttttatttaacttttcttttggacttttgggtagttgtttttttttgttttgttttgtttttttgagaaacagctacagctttgggtcatttttaactactgtattcccacaaggaatccccagatatttatgtatcttgatgttcagacatttatgtgttgataattttttaattatttaaatgtacttatattaagaaaaatatcaagtactacattttcttttgttcttgatagtagccaaagttaaatgtatcacattgaagaaggctagaaaaaaagaatgagtaatgtgatcgcttggttatccagaagtattgtttacattaaactccctttcatgttaatcaaacaagtgagtagctcacgcagcaacgtttttaataggatttttagacactgagggtcactccaaggatcagaagtatggaattttctgccaggctcaacaagggtctcatatctaacttcctccttaaaacagagaaggtcaatctagttccagagggttgaggcaggtgccaataattacatctttggagaggatttgatttctgcccagggatttgctcaccccaaggtcatctgataatttcacagatgctgtgtaacagaacacagccaaagtaaactgtgtaggggagccacatttacataggaaccaaatcaatgaatttaggggttacgattatagcaatttaagggcccaccagaagcaggcctcgaggagtcaatttgcctctgtgtgcctcagtggagacaagtgggaaaacatggtcccacctgtgcgagaccccctgtcctgtgctgctcactcaacaacatctttgtgttgctttcaccaggctgagaccctaccctatggggtatatgggcttttacctgtgcaccagtgtgacaggaaagattcatgtcactactgtccgtggctacaattcaaaggtatccaatgtcgctgtaaattttatggcactatttttattggaggatttggtcagaatgcagttgttgtacaactcataaatactaactgctgattttgacacatgtgtgctccaaatgatctggtggttatttaacgtacctcttaaaattcgttgaaacgatttcaggtcaactctgaagagtatttgaaagcaggacttcagaacagtgtttgatttttattttataaatttaagcattcaaattaggcaaatctttggctgcaggcagcaaaaacagctggacttatttaaaacaacttgtttttgagttttcttatatatatattgattatttgttttacacacatgcagtagcactttggtaagagttaaagagtaaagcagcttatgttgtcaggtcgttcttatctagagaagagctatagcagatctcggacaaactcagaatatattcactttcatttttgacaggattccctccacaactcagtttcatatattattccgtattacatttttgcagctaaattaccataaaatgtcagcaaatgtaaaaatttaatttctgaaaagcaccattagcccatttcccccaaattaaacgtaaatgttttttttcagcacatgttaccatgtctgacctgcaaaaatgctggagaaaaatgaaggaaaaaattatgtttttcagtttaattctgttaactgaagatattccaactcaaaaccagcctcatgctctgattagataatcttttacattgaacctttactctcaaagccatgtgtggagggggcttgtcactattgtaggctcactggattggtcatttagagtttcacagactcttaccagcatatatagtatttaattgtttcaaaaaaaatcaaactgtagttgttttggcgataggtctcacgcaacacatttttgtatgtgtgtgtgtgtgcgtgtgtgtgtgtgtgtgtgaaaaattgcattcattgacttcaggtagattaaggtatctttttattcattgccctcaggaaagttaaggtatcaatgagacccttaagccaatcatgtaataactgcatgtgtctggtccaggagaagtattgaataagccatttctactgcttactcatgtccctatttatgatttcaacatggatacatatttcagttctttctttttctcactatctgaaaatacatttccctccctctcttccccccaatatctccctttttttctctcttcctctatcttccaaaccccactttctccctcctccttttcctgtgttctcttaagcagatagcacatacccccacccagtaccaaatttcagaacacaagaaggtccagttcttcccccttcacataaaggaacatggtttgtcagcctttctcctgtttatgggtttcttccagcagaacagagacattgccaaccatattggatctgcttgctgtccaaaccagcaaactttcctgggcaaatcacaatcagtgagtaaatagacagcctttctgctgccttgggtttctgtgcagataaacagaaatgctctgattagaaaggaaatgaatggttccactcaaatgtcctgcaatttaggattgcagatttctgccttgaaatacctgtttctttgggacattccgtcctgatgatttttatttttgttggtttttatttttggggggaatgacatgtttgggtcttttatacatgaaaatttgtttgacaataatctcacaaaacatattttacatctgaacaaaatgcctttttgtttaccgtagcgtatacatttgttttgggatttttgtgtgtttgttgggaattttgtttttagccaggtcagtattgatgaggctgatcatttggctctttttttccttccagaagagttgcatcaacaaagttaattgtatttatgtatgtaaatagattttaagcttcattataaaatattgttaatgcctataactttttttcaatttttttgtgtgtgtttctaaggactttttcttaggtttgctaaatactgtagggaaaaaaatgcttctttctactttgtttattttagactttaaaatgagctacttcttattcacttttgtaaacagctaatagcatggttccaattttttttaagttcactttttttgttctaggggaaatgaatgtgcaaaaaaagaaaaagaactgttggttatttgtgttattctggatgtataaaaatcaatggaaaaaaataaactttcaaattgaaatgacggtataacacatctactgaaaaagcaacgggaaatgtggtcctatttaagccagcccccacctagggtctatttgtgtggcagttattgggtttggtcacaaaacatcctgaaaattcgtgcgtgggcttctttctccctggtacaaacgtatggaatgcttcttaaaggggaactgtcaagctggtgtcttcagccagatgacatgagagaatatcccagaaccctctctccaaggtgtttctagatagcacaggagagcaggcactgcactgtccacagtccacggtacacagtcgggtgggccgcctcccctctcctgggagcattcgtcgtgcccagcctgagcagggcagctggactgctgctgttcaggagccaccagagccttcctctctttgtaccacagtttcttctgtaaatccagtgttacaatcagtgtgaatggcaaataaacagtttgacaagtacatacaccata

SEQ ID NO: 16 - DNA, 1452 bp, Artificial Sequence
  RUNX1 cDNA sequence
acagttaaatttgtaatttgggttgtgtgaaaacttctttgggcctcataaacaaccacagaaccacaagttgggtagcctggcagtgtcagaagtctgaacccagcatagtggtcagcaggcaggacgaatcacactgaatgcaaaccacagggtttcgcagcgtggtaaaagaaatcattgagtcccccgccttcagaagagggtgcattttcaggaggaagcgatggcttcagacagcatatttgagtcatttccttcgtacccacagtgcttcatgagagaatgcatacttggaatgaatccttctagagacgtccacgatgccagcacgagccgccgcttcacgccgccttccaccgcgctgagcccaggcaagatgagcgaggcgttgccgctgggcgccccggacgccggcgctgccctggccggcaagctgaggagcggcgaccgcagcatggtggaggtgctggccgaccacccgggcgagctggtgcgcaccgacagccccaacttcctctgctccgtgctgcctacgcactggcgctgcaacaagaccctgcccatcgctttcaaggtggtggccctaggggatgttccagatggcactctggtcactgtgatggctggcaatgatgaaaactactcggctgagctgagaaatgctaccgcagccatgaagaaccaggttgcaagatttaatgacctcaggtttgtcggtcgaagtggaagagggaaaagcttcactctgaccatcactgtcttcacaaacccaccgcaagtcgccacctaccacagagccatcaaaatcacagtggatgggccccgagaacctcgaagacatcggcagaaactagatgatcagaccaagcccgggagcttgtccttttccgagcggctcagtgaactggagcagctgcggcgcacagccatgagggtcagcccacaccacccagcccccacgcccaaccctcgtgcctccctgaaccactccactgcctttaaccctcagcctcagagtcagatgcaggaggaagacacagcaccctggagatgttaaggcagaagtcagttcttctgtccatccctctccccagccaggatagagctatcttttccatctcatcctcagaagagactcagaagaaagatgacagccctcagaatgcacgttatgaggaaggcagaatgtgggtctgtaattcctccgtgtcccttctccccctctgcaaaccgtcgtaacaataatagttcctaacacatgggacaattgtgaggattaaatgagttagcctgcagaaatcacttgatgcacagcacatgggaagcattgtgtgtatttattaatccttcacaaagtctttgagatatatttttatcaaatatttagcatggatcccggtacactttcaatacttaataaatggtcaatgttattctttttcactatta

SEQ ID NO: 17 - DNA, 4693 bp, Artificial Sequence
  RUNX1 cDNA sequence
acagttaaatttgtaatttgggttgtgtgaaaacttctttgggcctcataaacaaccacagaaccacaagttgggtagcctggcagtgtcagaagtctgaacccagcatagtggtcagcaggcaggacgaatcacactgaatgcaaaccacagggtttcgcagcgtggtaaaagaaatcattgagtcccccgccttcagaagagggtgcattttcaggaggaagcgatggcttcagacagcatatttgagtcatttccttcgtacccacagtgcttcatgagagaatgcatacttggaatgaatccttctagagacgtccacgatgccagcacgagccgccgcttcacgccgccttccaccgcgctgagcccaggcaagatgagcgaggcgttgccgctgggcgccccggacgccggcgctgccctggccggcaagctgaggagcggcgaccgcagcatggtggaggtgctggccgaccacccgggcgagctggtgcgcaccgacagccccaacttcctctgctccgtgctgcctacgcactggcgctgcaacaagaccctgcccatcgctttcaaggtggtggccctaggggatgttccagatggcactctggtcactgtgatggctggcaatgatgaaaactactcggctgagctgagaaatgctaccgcagccatgaagaaccaggttgcaagatttaatgacctcaggtttgtcggtcgaagtggaagagggaaaagcttcactctgaccatcactgtcttcacaaacccaccgcaagtcgccacctaccacagagccatcaaaatcacagtggatgggccccgagaacctcgaagacatcggcagaaactagatgatcagaccaagcccgggagcttgtccttttccgagcggctcagtgaactggagcagctgcggcgcacagccatgagggtcagcccacaccacccagcccccacgcccaaccctcgtgcctccctgaaccactccactgcctttaaccctcagcctcagagtcagatgcaggatacaaggcagatccaaccatccccaccgtggtcctacgatcagtcctaccaatacctgggatccattgcctctccttctgtgcacccagcaacgcccatttcacctggacgtgccagcggcatgacaaccctctctgcagaactttccagtcgactctcaaacagttgtgattacttcaggtttcaccagatgccttagctgctgttcagagcttcacagaatgccttctaagagcttcacaacggcagtactattgacatttggggccaaataattctttgttggggggggtctgtcctgagcatcggagaatatttagcagcatccttggcctctagatgccaatagcatccccctcaccccagttaggacaataaaaaatgtttccagacattgccaaatttcccaaggggcaaaactgtccccaggtgagaaccactgccttccagtgttcttgggtggtacagtaaaataggaaaaccaacttaagtgcttggttttcacattacttttggccattaatgccaatattttcatggtacattctgctccaaggcattgagagtagcacaggtatcttggcatcttgtttagcttgtggtttctagaagcttatccctcaagaacaaaggcacttgtcagcttttactgattgttctcagggcacccctctgcacaccggctacggtcttcacctgaaataatgcctgttctccttcaaatgttcctgctatgggtctatcctttggaatttattacataagtcttttgacttggtcatcacccaagatcagcaccttatagtccaagaaccctaggggccaactcctccagctgactggtgttcagatggtagggtgactttttaaataaaaggaatgagtaacatgtgcactccaaagtcccatatcacagttacatttgtgaatatcctggacttcaatcacccaaggagtaagagagaacattttatggcatgggagtgtgaagtagataaaaaccatgcctcatttcagaacccaagaatgattcttttctttttggagggaggacagaattccagatgagctttcacagtggcatagaacagtatgggagactgctcttcaatttggcagaactccctctgagaaatcaagcctggagcacaggcctgaaaagtgttgtcataaacctggaggcaggaggggggtggaatacataaaaggaaagtggctgcctggccgacagctttgagaacctgacactgctctgtggctgctttgccttttaatccagcccgacagctttgtgctctgcccctcttcccggccccagccccacctgggcttccttctgcgctggggacttggactctgtctgtctctctctctctatcctttgcagacagactccacaccttgtctgaaaagagttgtcatctagaggtttacttttttttttctttttcaaaaaaaattaatgtttagctgccaacctgggcgacagacagcatgcattaatctgagtcatgcaaaagctccttttaaggcagccattacctgctcaggttgtttaatcctctgggggcagtaggaggggccctgtagcgaggctgctttcatccatgtcaagctggagagcgaagacttgagctgtcatggcaaatatttagccccatcaatgggaaaacacttccaaccaaaatacctggacctcctaagccccagatttcctactcttaaaaactctctgtgaatatcaggggatcccaactccccccacacttctgctgaatcaggggacaccaggccagccaaaaggacagaagagctacagctggatgggtgaactgcgcagactgatgggtttgaataagggatctgagacaagacacaaagatgaaaaccaacatttgaatatagcatttgaatctgagcatatctagaaggcctaagatattgtattatcaaaatgtgtgtaaaaaagatagtttgaccaaatggatggtcttttgtagtatgacgttgctcatgtgtacatagaagaaggatcacaggcagcattgcagctctttcttttggatgttctcctcacaagtgaaagaactattttcccccaacagctgagaccataacatcattccagtacttatgtccatgacaaatcacggactcactctggattccagtaacttggtaccatcaccacattaccatgtagtagttggaacctactggcagagcatgtccagacattgctgtaaaacagggtgacctttcgttcattttccagtggattcacctttttgtctcagggcaaatgaagcaagaggaataatgggcagagtcatttatttgtgtccagagtattgcatcagatgacaacaaactgactgtatttgcctaatgcttttcctcctgtcccagcttctccgtagactctataaatctaaatggaaaaatggagtaaagcttcctgttaactctcaaacatgtcacagctctccatgtcagcaaaaacaagtgacacagggcttgctcacagatggccccaaagagcgggcagggatgaaccctgtggaatgaggtgtggcctggctcgagaatgactagagtgtggccaaggaagggcagcctcagaaccactgtccgtttacaacgttttccctgcccacatgtctgcctggctttgaaaagattaacaggagtgtttgtttgaaagtcagactcctggtttcctcattagtgaagggatctgctacagacttgggctgtttctataaactttaattacctctgatgaggagtgtatcccctcatcacattcaccccaaaggtacagaggagttcatttttaaaaatgtgttagagcaataaaaggccattagagggagggaggatggggtgtggaagagacgagagagcgagcgagagagagagaaaacacactagctctccctgctggaataataggcttgaaatatgaggaagttgatcaactgccgctgccttccaaaaacagattaatccaccttggtagctttcctttcagagcaagcttttggctctgtcgactttctctatcagcctgaactcaaaaggacacaggccacatgccatctgagcttaagagttattttgtgtgttgatctgagaacttcacattttaaaacaatgaattcatgtttctactgtttgttgctgtctgtggatttgctgatataaagaggagagtcctagcctggtcatttaatgaataattctaaggaacctgaacttctccagggtgcccttctacatctgcagtggtggttctcagctggggtgactttgcttccgtcaccccacccgcaggatatctggcaatgtctggagacattctgagttgtcacaagaggggcgggcgatgctactaacacctaatgggtaaagcagagatgctgccacacatcctacgatgaacgagacagccccctccaccccagcaaatcatgatctggcccaaaatgtcaacagtgtcaacagttgagaaactctgatctacagatatagggaaccctgcctaatacacaaatcctccgtagttcccaagggcggcctgtagcggcacccgacctgacagcgttcagcgacccgcgccagttccccgcgctgccctccatctccgacccccgcatgc

SEQ ID NO: 18 - DNA, 5772 bp, Artificial Sequence
  RUNX1 cDNA sequence
acagttaaatttgtaatttgggttgtgtgaaaacttctttgggcctcataaacaaccacagaaccacaagttgggtagcctggcagtgtcagaagtctgaacccagcatagtggtcagcaggcaggacgaatcacactgaatgcaaaccacagggtttcgcagcgtggtaaaagaaatcattgagtcccccgccttcagaagagggtgcattttcaggaggaagcgatggcttcagacagcatatttgagtcatttccttcgtacccacagtgcttcatgagagatgccagcacgagccgccgcttcacgccgccttccaccgcgctgagcccaggcaagatgagcgaggcgttgccgctgggcgccccggacgccggcgctgccctggccggcaagctgaggagcggcgaccgcagcatggtggaggtgctggccgaccacccgggcgagctggtgcgcaccgacagccccaacttcctctgctccgtgctgcctacgcactggcgctgcaacaagaccctgcccatcgctttcaaggtggtggccctaggggatgttccagatggcactctggtcactgtgatggctggcaatgatgaaaactactcggctgagctgagaaatgctaccgcagccatgaagaaccaggttgcaagatttaatgacctcaggtttgtcggtcgaagtggaagagggaaaagcttcactctgaccatcactgtcttcacaaacccaccgcaagtcgccacctaccacagagccatcaaaatcacagtggatgggccccgagaacctcgaaatacaaggcagatccaaccatccccaccgtggtcctacgatcagtcctaccaatacctgggatccattgcctctccttctgtgcacccagcaacgcccatttcacctggacgtgccagcggcatgacaaccctctctgcagaactttccagtcgactctcaacggcacccgacctgacagcgttcagcgacccgcgccagttccccgcgctgccctccatctccgacccccgcatgcactatccaggcgccttcacctactccccgacgccggtcacctcgggcatcggcatcggcatgtcggccatgggctcggccacgcgctaccacacctacctgccgccgccctaccccggctcgtcgcaagcgcagggaggcccgttccaagccagctcgccctcctaccacctgtactacggcgcctcggccggctcctaccagttctccatggtgggcggcgagcgctcgccgccgcgcatcctgccgccctgcaccaacgcctccaccggctccgcgctgctcaaccccagcctcccgaaccagagcgacgtggtggaggccgagggcagccacagcaactcccccaccaacatggcgccctccgcgcgcctggaggaggccgtgtggaggccctactgaggcgccaggcctggcccggctgggccccgcgggccgccgccttcgcctccgggcgcgcgggcctcctgttcgcgacaagcccgccgggatcccgggccctgggcccggccaccgtcctggggccgagggcgcccgacggccaggatctcgctgtaggtcaggcccgcgcagcctcctgcgcccagaagcccacgccgccgccgtctgctggcgccccggccctcgcggaggtgtccgaggcgacgcacctcgagggtgtccgccggccccagcacccaggggacgcgctggaaagcaaacaggaagattcccggagggaaactgtgaatgcttctgatttagcaatgctgtgaataaaaagaaagattttatacccttgacttaactttttaaccaagttgtttattccaaagagtgtggaattttggttggggtggggggagaggagggatgcaactcgccctgtttggcatctaattcttatttttaatttttccgcaccttatcaattgcaaaatgcgtatttgcatttgggtggtttttatttttatatacgtttatataaatatatataaattgagcttgcttctttcttgctttgaccatggaaagaaatatgattcccttttctttaagttttatttaacttttcttttggacttttgggtagttgtttttttttgttttgttttgtttttttgagaaacagctacagctttgggtcatttttaactactgtattcccacaaggaatccccagatatttatgtatcttgatgttcagacatttatgtgttgataattttttaattatttaaatgtacttatattaagaaaaatatcaagtactacattttcttttgttcttgatagtagccaaagttaaatgtatcacattgaagaaggctagaaaaaaagaatgagtaatgtgatcgcttggttatccagaagtattgtttacattaaactccctttcatgttaatcaaacaagtgagtagctcacgcagcaacgtttttaataggatttttagacactgagggtcactccaaggatcagaagtatggaattttctgccaggctcaacaagggtctcatatctaacttcctccttaaaacagagaaggtcaatctagttccagagggttgaggcaggtgccaataattacatctttggagaggatttgatttctgcccagggatttgctcaccccaaggtcatctgataatttcacagatgctgtgtaacagaacacagccaaagtaaactgtgtaggggagccacatttacataggaaccaaatcaatgaatttaggggttacgattatagcaatttaagggcccaccagaagcaggcctcgaggagtcaatttgcctctgtgtgcctcagtggagacaagtgggaaaacatggtcccacctgtgcgagaccccctgtcctgtgctgctcactcaacaacatctttgtgttgctttcaccaggctgagaccctaccctatggggtatatgggcttttacctgtgcaccagtgtgacaggaaagattcatgtcactactgtccgtggctacaattcaaaggtatccaatgtcgctgtaaattttatggcactatttttattggaggatttggtcagaatgcagttgttgtacaactcataaatactaactgctgattttgacacatgtgtgctccaaatgatctggtggttatttaacgtacctcttaaaattcgttgaaacgatttcaggtcaactctgaagagtatttgaaagcaggacttcagaacagtgtttgatttttattttataaatttaagcattcaaattaggcaaatctttggctgcaggcagcaaaaacagctggacttatttaaaacaacttgtttttgagttttcttatatatatattgattatttgttttacacacatgcagtagcactttggtaagagttaaagagtaaagcagcttatgttgtcaggtcgttcttatctagagaagagctatagcagatctcggacaaactcagaatatattcactttcatttttgacaggattccctccacaactcagtttcatatattattccgtattacatttttgcagctaaattaccataaaatgtcagcaaatgtaaaaatttaatttctgaaaagcaccattagcccatttcccccaaattaaacgtaaatgttttttttcagcacatgttaccatgtctgacctgcaaaaatgctggagaaaaatgaaggaaaaaattatgtttttcagtttaattctgttaactgaagatattccaactcaaaaccagcctcatgctctgattagataatcttttacattgaacctttactctcaaagccatgtgtggagggggcttgtcactattgtaggctcactggattggtcatttagagtttcacagactcttaccagcatatatagtatttaattgtttcaaaaaaaatcaaactgtagttgttttggcgataggtctcacgcaacacatttttgtatgtgtgtgtgtgtgcgtgtgtgtgtgtgtgtgtgaaaaattgcattcattgacttcaggtagattaaggtatctttttattcattgccctcaggaaagttaaggtatcaatgagacccttaagccaatcatgtaataactgcatgtgtctggtccaggagaagtattgaataagccatttctactgcttactcatgtccctatttatgatttcaacatggatacatatttcagttctttctttttctcactatctgaaaatacatttccctccctctcttccccccaatatctccctttttttctctcttcctctatcttccaaaccccactttctccctcctccttttcctgtgttctcttaagcagatagcacatacccccacccagtaccaaatttcagaacacaagaaggtccagttcttcccccttcacataaaggaacatggtttgtcagcctttctcctgtttatgggtttcttccagcagaacagagacattgccaaccatattggatctgcttgctgtccaaaccagcaaactttcctgggcaaatcacaatcagtgagtaaatagacagcctttctgctgccttgggtttctgtgcagataaacagaaatgctctgattagaaaggaaatgaatggttccactcaaatgtcctgcaatttaggattgcagatttctgccttgaaatacctgtttctttgggacattccgtcctgatgatttttatttttgttggtttttatttttggggggaatgacatgtttgggtcttttatacatgaaaatttgtttgacaataatctcacaaaacatattttacatctgaacaaaatgcctttttgtttaccgtagcgtatacatttgttttgggatttttgtgtgtttgttgggaattttgtttttagccaggtcagtattgatgaggctgatcatttggctctttttttccttccagaagagttgcatcaacaaagttaattgtatttatgtatgtaaatagattttaagcttcattataaaatattgttaatgcctataactttttttcaatttttttgtgtgtgtttctaaggactttttcttaggtttgctaaatactgtagggaaaaaaatgcttctttctactttgtttattttagactttaaaatgagctacttcttattcacttttgtaaacagctaatagcatggttccaattttttttaagttcactttttttgttctaggggaaatgaatgtgcaaaaaaagaaaaagaactgttggttatttgtgttattctggatgtataaaaatcaatggaaaaaaataaactttcaaattgaaatgacggtataacacatctactgaaaaagcaacgggaaatgtggtcctatttaagccagcccccacctagggtctatttgtgtggcagttattgggtttggtcacaaaacatcctgaaaattcgtgcgtgggcttctttctccctggtacaaacgtatggaatgcttcttaaaggggaactgtcaagctggtgtcttcagccagatgacatgagagaatatcccagaaccctctctccaaggtgtttctagatagcacaggagagcaggcactgcactgtccacagtccacggtacacagtcgggtgggccgcctcccctctcctgggagcattcgtcgtgcccagcctgagcagggcagctggactgctgctgttcaggagccaccagagccttcctctctttgtaccacagtttcttctgtaaatccagtgttacaatcagtgtgaatggcaaataaacagtttgacaagtacatacaccata

SEQ ID NO: 19 - DNA, 5811 bp, Artificial Sequence
  RUNX1 cDNA sequence
acagttaaatttgtaatttgggttgtgtgaaaacttctttgggcctcataaacaaccacagaaccacaagttgggtagcctggcagtgtcagaagtctgaacccagcatagtggtcagcaggcaggacgaatcacactgaatgcaaaccacagggtttcgcagcgtggtaaaagaaatcattgagtcccccgccttcagaagagggtgcattttcaggaggaagcgatggcttcagacagcatatttgagtcatttccttcgtacccacagtgcttcatgagagaatgcatacttggaatgaatccttctagagacgtccacgatgccagcacgagccgccgcttcacgccgccttccaccgcgctgagcccaggcaagatgagcgaggcgttgccgctgggcgccccggacgccggcgctgccctggccggcaagctgaggagcggcgaccgcagcatggtggaggtgctggccgaccacccgggcgagctggtgcgcaccgacagccccaacttcctctgctccgtgctgcctacgcactggcgctgcaacaagaccctgcccatcgctttcaaggtggtggccctaggggatgttccagatggcactctggtcactgtgatggctggcaatgatgaaaactactcggctgagctgagaaatgctaccgcagccatgaagaaccaggttgcaagatttaatgacctcaggtttgtcggtcgaagtggaagagggaaaagcttcactctgaccatcactgtcttcacaaacccaccgcaagtcgccacctaccacagagccatcaaaatcacagtggatgggccccgagaacctcgaaatacaaggcagatccaaccatccccaccgtggtcctacgatcagtcctaccaatacctgggatccattgcctctccttctgtgcacccagcaacgcccatttcacctggacgtgccagcggcatgacaaccctctctgcagaactttccagtcgactctcaacggcacccgacctgacagcgttcagcgacccgcgccagttccccgcgctgccctccatctccgacccccgcatgcactatccaggcgccttcacctactccccgacgccggtcacctcgggcatcggcatcggcatgtcggccatgggctcggccacgcgctaccacacctacctgccgccgccctaccccggctcgtcgcaagcgcagggaggcccgttccaagccagctcgccctcctaccacctgtactacggcgcctcggccggctcctaccagttctccatggtgggcggcgagcgctcgccgccgcgcatcctgccgccctgcaccaacgcctccaccggctccgcgctgctcaaccccagcctcccgaaccagagcgacgtggtggaggccgagggcagccacagcaactcccccaccaacatggcgccctccgcgcgcctggaggaggccgtgtggaggccctactgaggcgccaggcctggcccggctgggccccgcgggccgccgccttcgcctccgggcgcgcgggcctcctgttcgcgacaagcccgccgggatcccgggccctgggcccggccaccgtcctggggccgagggcgcccgacggccaggatctcgctgtaggtcaggcccgcgcagcctcctgcgcccagaagcccacgccgccgccgtctgctggcgccccggccctcgcggaggtgtccgaggcgacgcacctcgagggtgtccgccggccccagcacccaggggacgcgctggaaagcaaacaggaagattcccggagggaaactgtgaatgcttctgatttagcaatgctgtgaataaaaagaaagattttatacccttgacttaactttttaaccaagttgtttattccaaagagtgtggaattttggttggggtggggggagaggagggatgcaactcgccctgtttggcatctaattcttatttttaatttttccgcaccttatcaattgcaaaatgcgtatttgcatttgggtggtttttatttttatatacgtttatataaatatatataaattgagcttgcttctttcttgctttgaccatggaaagaaatatgattcccttttctttaagttttatttaacttttcttttggacttttgggtagttgtttttttttgttttgttttgtttttttgagaaacagctacagctttgggtcatttttaactactgtattcccacaaggaatccccagatatttatgtatcttgatgttcagacatttatgtgttgataattttttaattatttaaatgtacttatattaagaaaaatatcaagtactacattttcttttgttcttgatagtagccaaagttaaatgtatcacattgaagaaggctagaaaaaaagaatgagtaatgtgatcgcttggttatccagaagtattgtttacattaaactccctttcatgttaatcaaacaagtgagtagctcacgcagcaacgtttttaataggatttttagacactgagggtcactccaaggatcagaagtatggaattttctgccaggctcaacaagggtctcatatctaacttcctccttaaaacagagaaggtcaatctagttccagagggttgaggcaggtgccaataattacatctttggagaggatttgatttctgcccagggatttgctcaccccaaggtcatctgataatttcacagatgctgtgtaacagaacacagccaaagtaaactgtgtaggggagccacatttacataggaaccaaatcaatgaatttaggggttacgattatagcaatttaagggcccaccagaagcaggcctcgaggagtcaatttgcctctgtgtgcctcagtggagacaagtgggaaaacatggtcccacctgtgcgagaccccctgtcctgtgctgctcactcaacaacatctttgtgttgctttcaccaggctgagaccctaccctatggggtatatgggcttttacctgtgcaccagtgtgacaggaaagattcatgtcactactgtccgtggctacaattcaaaggtatccaatgtcgctgtaaattttatggcactatttttattggaggatttggtcagaatgcagttgttgtacaactcataaatactaactgctgattttgacacatgtgtgctccaaatgatctggtggttatttaacgtacctcttaaaattcgttgaaacgatttcaggtcaactctgaagagtatttgaaagcaggacttcagaacagtgtttgatttttattttataaatttaagcattcaaattaggcaaatctttggctgcaggcagcaaaaacagctggacttatttaaaacaacttgtttttgagttttcttatatatatattgattatttgttttacacacatgcagtagcactttggtaagagttaaagagtaaagcagcttatgttgtcaggtcgttcttatctagagaagagctatagcagatctcggacaaactcagaatatattcactttcatttttgacaggattccctccacaactcagtttcatatattattccgtattacatttttgcagctaaattaccataaaatgtcagcaaatgtaaaaatttaatttctgaaaagcaccattagcccatttcccccaaattaaacgtaaatgttttttttcagcacatgttaccatgtctgacctgcaaaaatgctggagaaaaatgaaggaaaaaattatgtttttcagtttaattctgttaactgaagatattccaactcaaaaccagcctcatgctctgattagataatcttttacattgaacctttactctcaaagccatgtgtggagggggcttgtcactattgtaggctcactggattggtcatttagagtttcacagactcttaccagcatatatagtatttaattgtttcaaaaaaaatcaaactgtagttgttttggcgataggtctcacgcaacacatttttgtatgtgtgtgtgtgtgcgtgtgtgtgtgtgtgtgtgaaaaattgcattcattgacttcaggtagattaaggtatctttttattcattgccctcaggaaagttaaggtatcaatgagacccttaagccaatcatgtaataactgcatgtgtctggtccaggagaagtattgaataagccatttctactgcttactcatgtccctatttatgatttcaacatggatacatatttcagttctttctttttctcactatctgaaaatacatttccctccctctcttccccccaatatctccctttttttctctcttcctctatcttccaaaccccactttctccctcctccttttcctgtgttctcttaagcagatagcacatacccccacccagtaccaaatttcagaacacaagaaggtccagttcttcccccttcacataaaggaacatggtttgtcagcctttctcctgtttatgggtttcttccagcagaacagagacattgccaaccatattggatctgcttgctgtccaaaccagcaaactttcctgggcaaatcacaatcagtgagtaaatagacagcctttctgctgccttgggtttctgtgcagataaacagaaatgctctgattagaaaggaaatgaatggttccactcaaatgtcctgcaatttaggattgcagatttctgccttgaaatacctgtttctttgggacattccgtcctgatgatttttatttttgttggtttttatttttggggggaatgacatgtttgggtcttttatacatgaaaatttgtttgacaataatctcacaaaacatattttacatctgaacaaaatgcctttttgtttaccgtagcgtatacatttgttttgggatttttgtgtgtttgttgggaattttgtttttagccaggtcagtattgatgaggctgatcatttggctctttttttccttccagaagagttgcatcaacaaagttaattgtatttatgtatgtaaatagattttaagcttcattataaaatattgttaatgcctataactttttttcaatttttttgtgtgtgtttctaaggactttttcttaggtttgctaaatactgtagggaaaaaaatgcttctttctactttgtttattttagactttaaaatgagctacttcttattcacttttgtaaacagctaatagcatggttccaattttttttaagttcactttttttgttctaggggaaatgaatgtgcaaaaaaagaaaaagaactgttggttatttgtgttattctggatgtataaaaatcaatggaaaaaaataaactttcaaattgaaatgacggtataacacatctactgaaaaagcaacgggaaatgtggtcctatttaagccagcccccacctagggtctatttgtgtggcagttattgggtttggtcacaaaacatcctgaaaattcgtgcgtgggcttctttctccctggtacaaacgtatggaatgcttcttaaaggggaactgtcaagctggtgtcttcagccagatgacatgagagaatatcccagaaccctctctccaaggtgtttctagatagcacaggagagcaggcactgcactgtccacagtccacggtacacagtcgggtgggccgcctcccctctcctgggagcattcgtcgtgcccagcctgagcagggcagctggactgctgctgttcaggagccaccagagccttcctctctttgtaccacagtttcttctgtaaatccagtgttacaatcagtgtgaatggcaaataaacagtttgacaagtacatacaccata

SEQ ID NO: 20 - DNA, 5772 bp, Artificial Sequence
  RUNX1 cDNA sequence
cactttttaatgcactaagcaatcggttgctaggagcccatcctgggtcagaggccgatccgcagaaccagaacgttttcccctcctggactatgccagcacgagccgccgcttcacgccgccttccaccgcgctgagcccaggcaagatgagcgaggcgttgccgctgggcgccccggacgccggcgctgccctggccggcaagctgaggagcggcgaccgcagcatggtggaggtgctggccgaccacccgggcgagctggtgcgcaccgacagccccaacttcctctgctccgtgctgcctacgcactggcgctgcaacaagaccctgcccatcgctttcaaggtggtggccctaggggatgttccagatggcactctggtcactgtgatggctggcaatgatgaaaactactcggctgagctgagaaatgctaccgcagccatgaagaaccaggttgcaagatttaatgacctcaggtttgtcggtcgaagtggaagagggaaaagcttcactctgaccatcactgtcttcacaaacccaccgcaagtcgccacctaccacagagccatcaaaatcacagtggatgggccccgagaacctcgaagacatcggcagaaactagatgatcagaccaagcccgggagcttgtccttttccgagcggctcagtgaactggagcagctgcggcgcacagccatgagggtcagcccacaccacccagcccccacgcccaaccctcgtgcctccctgaaccactccactgcctttaaccctcagcctcagagtcagatgcaggatacaaggcagatccaaccatccccaccgtggtcctacgatcagtcctaccaatacctgggatccattgcctctccttctgtgcacccagcaacgcccatttcacctggacgtgccagcggcatgacaaccctctctgcagaactttccagtcgactctcaacggcacccgacctgacagcgttcagcgacccgcgccagttccccgcgctgccctccatctccgacccccgcatgcactatccaggcgccttcacctactccccgacgccggtcacctcgggcatcggcatcggcatgtcggccatgggctcggccacgcgctaccacacctacctgccgccgccctaccccggctcgtcgcaagcgcagggaggcccgttccaagccagctcgccctcctaccacctgtactacggcgcctcggccggctcctaccagttctccatggtgggcggcgagcgctcgccgccgcgcatcctgccgccctgcaccaacgcctccaccggctccgcgctgctcaaccccagcctcccgaaccagagcgacgtggtggaggccgagggcagccacagcaactcccccaccaacatggcgccctccgcgcgcctggaggaggccgtgtggaggccctactgaggcgccaggcctggcccggctgggccccgcgggccgccgccttcgcctccgggcgcgcgggcctcctgttcgcgacaagcccgccgggatcccgggccctgggcccggccaccgtcctggggccgagggcgcccgacggccaggatctcgctgtaggtcaggcccgcgcagcctcctgcgcccagaagcccacgccgccgccgtctgctggcgccccggccctcgcggaggtgtccgaggcgacgcacctcgagggtgtccgccggccccagcacccaggggacgcgctggaaagcaaacaggaagattcccggagggaaactgtgaatgcttctgatttagcaatgctgtgaataaaaagaaagattttatacccttgacttaactttttaaccaagttgtttattccaaagagtgtggaattttggttggggtggggggagaggagggatgcaactcgccctgtttggcatctaattcttatttttaatttttccgcaccttatcaattgcaaaatgcgtatttgcatttgggtggtttttatttttatatacgtttatataaatatatataaattgagcttgcttctttcttgctttgaccatggaaagaaatatgattcccttttctttaagttttatttaacttttcttttggacttttgggtagttgtttttttttgttttgttttgtttttttgagaaacagctacagctttgggtcatttttaactactgtattcccacaaggaatccccagatatttatgtatcttgatgttcagacatttatgtgttgataattttttaattatttaaatgtacttatattaagaaaaatatcaagtactacattttcttttgttcttgatagtagccaaagttaaatgtatcacattgaagaaggctagaaaaaaagaatgagtaatgtgatcgcttggttatccagaagtattgtttacattaaactccctttcatgttaatcaaacaagtgagtagctcacgcagcaacgtttttaataggatttttagacactgagggtcactccaaggatcagaagtatggaattttctgccaggctcaacaagggtctcatatctaacttcctccttaaaacagagaaggtcaatctagttccagagggttgaggcaggtgccaataattacatctttggagaggatttgatttctgcccagggatttgctcaccccaaggtcatctgataatttcacagatgctgtgtaacagaacacagccaaagtaaactgtgtaggggagccacatttacataggaaccaaatcaatgaatttaggggttacgattatagcaatttaagggcccaccagaagcaggcctcgaggagtcaatttgcctctgtgtgcctcagtggagacaagtgggaaaacatggtcccacctgtgcgagaccccctgtcctgtgctgctcactcaacaacatctttgtgttgctttcaccaggctgagaccctaccctatggggtatatgggcttttacctgtgcaccagtgtgacaggaaagattcatgtcactactgtccgtggctacaattcaaaggtatccaatgtcgctgtaaattttatggcactatttttattggaggatttggtcagaatgcagttgttgtacaactcataaatactaactgctgattttgacacatgtgtgctccaaatgatctggtggttatttaacgtacctcttaaaattcgttgaaacgatttcaggtcaactctgaagagtatttgaaagcaggacttcagaacagtgtttgatttttattttataaatttaagcattcaaattaggcaaatctttggctgcaggcagcaaaaacagctggacttatttaaaacaacttgtttttgagttttcttatatatatattgattatttgttttacacacatgcagtagcactttggtaagagttaaagagtaaagcagcttatgttgtcaggtcgttcttatctagagaagagctatagcagatctcggacaaactcagaatatattcactttcatttttgacaggattccctccacaactcagtttcatatattattccgtattacatttttgcagctaaattaccataaaatgtcagcaaatgtaaaaatttaatttctgaaaagcaccattagcccatttcccccaaattaaacgtaaatgttttttttcagcacatgttaccatgtctgacctgcaaaaatgctggagaaaaatgaaggaaaaaattatgtttttcagtttaattctgttaactgaagatattccaactcaaaaccagcctcatgctctgattagataatcttttacattgaacctttactctcaaagccatgtgtggagggggcttgtcactattgtaggctcactggattggtcatttagagtttcacagactcttaccagcatatatagtatttaattgtttcaaaaaaaatcaaactgtagttgttttggcgataggtctcacgcaacacatttttgtatgtgtgtgtgtgtgcgtgtgtgtgtgtgtgtgtgaaaaattgcattcattgacttcaggtagattaaggtatctttttattcattgccctcaggaaagttaaggtatcaatgagacccttaagccaatcatgtaataactgcatgtgtctggtccaggagaagtattgaataagccatttctactgcttactcatgtccctatttatgatttcaacatggatacatatttcagttctttctttttctcactatctgaaaatacatttccctccctctcttccccccaatatctccctttttttctctcttcctctatcttccaaaccccactttctccctcctccttttcctgtgttctcttaagcagatagcacatacccccacccagtaccaaatttcagaacacaagaaggtccagttcttcccccttcacataaaggaacatggtttgtcagcctttctcctgtttatgggtttcttccagcagaacagagacattgccaaccatattggatctgcttgctgtccaaaccagcaaactttcctgggcaaatcacaatcagtgagtaaatagacagcctttctgctgccttgggtttctgtgcagataaacagaaatgctctgattagaaaggaaatgaatggttccactcaaatgtcctgcaatttaggattgcagatttctgccttgaaatacctgtttctttgggacattccgtcctgatgatttttatttttgttggtttttatttttggggggaatgacatgtttgggtcttttatacatgaaaatttgtttgacaataatctcacaaaacatattttacatctgaacaaaatgcctttttgtttaccgtagcgtatacatttgttttgggatttttgtgtgtttgttgggaattttgtttttagccaggtcagtattgatgaggctgatcatttggctctttttttccttccagaagagttgcatcaacaaagttaattgtatttatgtatgtaaatagattttaagcttcattataaaatattgttaatgcctataactttttttcaatttttttgtgtgtgtttctaaggactttttcttaggtttgctaaatactgtagggaaaaaaatgcttctttctactttgtttattttagactttaaaatgagctacttcttattcacttttgtaaacagctaatagcatggttccaattttttttaagttcactttttttgttctaggggaaatgaatgtgcaaaaaaagaaaaagaactgttggttatttgtgttattctggatgtataaaaatcaatggaaaaaaataaactttcaaattgaaatgacggtataacacatctactgaaaaagcaacgggaaatgtggtcctatttaagccagcccccacctagggtctatttgtgtggcagttattgggtttggtcacaaaacatcctgaaaattcgtgcgtgggcttctttctccctggtacaaacgtatggaatgcttcttaaaggggaactgtcaagctggtgtcttcagccagatgacatgagagaatatcccagaaccctctctccaaggtgtttctagatagcacaggagagcaggcactgcactgtccacagtccacggtacacagtcgggtgggccgcctcccctctcctgggagcattcgtcgtgcccagcctgagcagggcagctggactgctgctgttcaggagccaccagagccttcctctctttgtaccacagtttcttctgtaaatccagtgttacaatcagtgtgaatggcaaataaacagtttgacaagtacatacaccata

SEQ ID NO: 21 - DNA, 5964 bp, Artificial Sequence
  RUNX1 cDNA sequence
acagttaaatttgtaatttgggttgtgtgaaaacttctttgggcctcataaacaaccacagaaccacaagttgggtagcctggcagtgtcagaagtctgaacccagcatagtggtcagcaggcaggacgaatcacactgaatgcaaaccacagggtttcgcagcgtggtaaaagaaatcattgagtcccccgccttcagaagagggtgcattttcaggaggaagcgatggcttcagacagcatatttgagtcatttccttcgtacccacagtgcttcatgagagatgccagcacgagccgccgcttcacgccgccttccaccgcgctgagcccaggcaagatgagcgaggcgttgccgctgggcgccccggacgccggcgctgccctggccggcaagctgaggagcggcgaccgcagcatggtggaggtgctggccgaccacccgggcgagctggtgcgcaccgacagccccaacttcctctgctccgtgctgcctacgcactggcgctgcaacaagaccctgcccatcgctttcaaggtggtggccctaggggatgttccagatggcactctggtcactgtgatggctggcaatgatgaaaactactcggctgagctgagaaatgctaccgcagccatgaagaaccaggttgcaagatttaatgacctcaggtttgtcggtcgaagtggaagagggaaaagcttcactctgaccatcactgtcttcacaaacccaccgcaagtcgccacctaccacagagccatcaaaatcacagtggatgggccccgagaacctcgaagacatcggcagaaactagatgatcagaccaagcccgggagcttgtccttttccgagcggctcagtgaactggagcagctgcggcgcacagccatgagggtcagcccacaccacccagcccccacgcccaaccctcgtgcctccctgaaccactccactgcctttaaccctcagcctcagagtcagatgcaggatacaaggcagatccaaccatccccaccgtggtcctacgatcagtcctaccaatacctgggatccattgcctctccttctgtgcacccagcaacgcccatttcacctggacgtgccagcggcatgacaaccctctctgcagaactttccagtcgactctcaacggcacccgacctgacagcgttcagcgacccgcgccagttccccgcgctgccctccatctccgacccccgcatgcactatccaggcgccttcacctactccccgacgccggtcacctcgggcatcggcatcggcatgtcggccatgggctcggccacgcgctaccacacctacctgccgccgccctaccccggctcgtcgcaagcgcagggaggcccgttccaagccagctcgccctcctaccacctgtactacggcgcctcggccggctcctaccagttctccatggtgggcggcgagcgctcgccgccgcgcatcctgccgccctgcaccaacgcctccaccggctccgcgctgctcaaccccagcctcccgaaccagagcgacgtggtggaggccgagggcagccacagcaactcccccaccaacatggcgccctccgcgcgcctggaggaggccgtgtggaggccctactgaggcgccaggcctggcccggctgggccccgcgggccgccgccttcgcctccgggcgcgcgggcctcctgttcgcgacaagcccgccgggatcccgggccctgggcccggccaccgtcctggggccgagggcgcccgacggccaggatctcgctgtaggtcaggcccgcgcagcctcctgcgcccagaagcccacgccgccgccgtctgctggcgccccggccctcgcggaggtgtccgaggcgacgcacctcgagggtgtccgccggccccagcacccaggggacgcgctggaaagcaaacaggaagattcccggagggaaactgtgaatgcttctgatttagcaatgctgtgaataaaaagaaagattttatacccttgacttaactttttaaccaagttgtttattccaaagagtgtggaattttggttggggtggggggagaggagggatgcaactcgccctgtttggcatctaattcttatttttaatttttccgcaccttatcaattgcaaaatgcgtatttgcatttgggtggtttttatttttatatacgtttatataaatatatataaattgagcttgcttctttcttgctttgaccatggaaagaaatatgattcccttttctttaagttttatttaacttttcttttggacttttgggtagttgtttttttttgttttgttttgtttttttgagaaacagctacagctttgggtcatttttaactactgtattcccacaaggaatccccagatatttatgtatcttgatgttcagacatttatgtgttgataattttttaattatttaaatgtacttatattaagaaaaatatcaagtactacattttcttttgttcttgatagtagccaaagttaaatgtatcacattgaagaaggctagaaaaaaagaatgagtaatgtgatcgcttggttatccagaagtattgtttacattaaactccctttcatgttaatcaaacaagtgagtagctcacgcagcaacgtttttaataggatttttagacactgagggtcactccaaggatcagaagtatggaattttctgccaggctcaacaagggtctcatatctaacttcctccttaaaacagagaaggtcaatctagttccagagggttgaggcaggtgccaataattacatctttggagaggatttgatttctgcccagggatttgctcaccccaaggtcatctgataatttcacagatgctgtgtaacagaacacagccaaagtaaactgtgtaggggagccacatttacataggaaccaaatcaatgaatttaggggttacgattatagcaatttaagggcccaccagaagcaggcctcgaggagtcaatttgcctctgtgtgcctcagtggagacaagtgggaaaacatggtcccacctgtgcgagaccccctgtcctgtgctgctcactcaacaacatctttgtgttgctttcaccaggctgagaccctaccctatggggtatatgggcttttacctgtgcaccagtgtgacaggaaagattcatgtcactactgtccgtggctacaattcaaaggtatccaatgtcgctgtaaattttatggcactatttttattggaggatttggtcagaatgcagttgttgtacaactcataaatactaactgctgattttgacacatgtgtgctccaaatgatctggtggttatttaacgtacctcttaaaattcgttgaaacgatttcaggtcaactctgaagagtatttgaaagcaggacttcagaacagtgtttgatttttattttataaatttaagcattcaaattaggcaaatctttggctgcaggcagcaaaaacagctggacttatttaaaacaacttgtttttgagttttcttatatatatattgattatttgttttacacacatgcagtagcactttggtaagagttaaagagtaaagcagcttatgttgtcaggtcgttcttatctagagaagagctatagcagatctcggacaaactcagaatatattcactttcatttttgacaggattccctccacaactcagtttcatatattattccgtattacatttttgcagctaaattaccataaaatgtcagcaaatgtaaaaatttaatttctgaaaagcaccattagcccatttcccccaaattaaacgtaaatgttttttttcagcacatgttaccatgtctgacctgcaaaaatgctggagaaaaatgaaggaaaaaattatgtttttcagtttaattctgttaactgaagatattccaactcaaaaccagcctcatgctctgattagataatcttttacattgaacctttactctcaaagccatgtgtggagggggcttgtcactattgtaggctcactggattggtcatttagagtttcacagactcttaccagcatatatagtatttaattgtttcaaaaaaaatcaaactgtagttgttttggcgataggtctcacgcaacacatttttgtatgtgtgtgtgtgtgcgtgtgtgtgtgtgtgtgtgaaaaattgcattcattgacttcaggtagattaaggtatctttttattcattgccctcaggaaagttaaggtatcaatgagacccttaagccaatcatgtaataactgcatgtgtctggtccaggagaagtattgaataagccatttctactgcttactcatgtccctatttatgatttcaacatggatacatatttcagttctttctttttctcactatctgaaaatacatttccctccctctcttccccccaatatctccctttttttctctcttcctctatcttccaaaccccactttctccctcctccttttcctgtgttctcttaagcagatagcacatacccccacccagtaccaaatttcagaacacaagaaggtccagttcttcccccttcacataaaggaacatggtttgtcagcctttctcctgtttatgggtttcttccagcagaacagagacattgccaaccatattggatctgcttgctgtccaaaccagcaaactttcctgggcaaatcacaatcagtgagtaaatagacagcctttctgctgccttgggtttctgtgcagataaacagaaatgctctgattagaaaggaaatgaatggttccactcaaatgtcctgcaatttaggattgcagatttctgccttgaaatacctgtttctttgggacattccgtcctgatgatttttatttttgttggtttttatttttggggggaatgacatgtttgggtcttttatacatgaaaatttgtttgacaataatctcacaaaacatattttacatctgaacaaaatgcctttttgtttaccgtagcgtatacatttgttttgggatttttgtgtgtttgttgggaattttgtttttagccaggtcagtattgatgaggctgatcatttggctctttttttccttccagaagagttgcatcaacaaagttaattgtatttatgtatgtaaatagattttaagcttcattataaaatattgttaatgcctataactttttttcaatttttttgtgtgtgtttctaaggactttttcttaggtttgctaaatactgtagggaaaaaaatgcttctttctactttgtttattttagactttaaaatgagctacttcttattcacttttgtaaacagctaatagcatggttccaattttttttaagttcactttttttgttctaggggaaatgaatgtgcaaaaaaagaaaaagaactgttggttatttgtgttattctggatgtataaaaatcaatggaaaaaaataaactttcaaattgaaatgacggtataacacatctactgaaaaagcaacgggaaatgtggtcctatttaagccagcccccacctagggtctatttgtgtggcagttattgggtttggtcacaaaacatcctgaaaattcgtgcgtgggcttctttctccctggtacaaacgtatggaatgcttcttaaaggggaactgtcaagctggtgtcttcagccagatgacatgagagaatatcccagaaccctctctccaaggtgtttctagatagcacaggagagcaggcactgcactgtccacagtccacggtacacagtcgggtgggccgcctcccctctcctgggagcattcgtcgtgcccagcctgagcagggcagctggactgctgctgttcaggagccaccagagccttcctctctttgtaccacagtttcttctgtaaatccagtgttacaatcagtgtgaatggcaaataaacagtttgacaagtacatacaccata

SEQ ID NO: 22 - DNA, 6078 bp, Artificial Sequence
  RUNX1 cDNA sequence
gtaatttgggttgtgtgaaaacttctttgggcctcataaacaaccacagaaccacaagttgggtagcctggcagtgtcagaagtctgaacccagcatagtggtcagcaggcaggacgaatcacactgaatgcaaaccacagggtttcgcagcgtggtgagcatcaccaacccacagccaaggcggcgctggctttttttttttttttaatctttaacaatttgaatatttgtttttacaaaggtaaaagaaatcattgagtcccccgccttcagaagagggtgcattttcaggaggaagcgatggcttcagacagcatatttgagtcatttccttcgtacccacagtgcttcatgagagaatgcatacttggaatgaatccttctagagacgtccacgatgccagcacgagccgccgcttcacgccgccttccaccgcgctgagcccaggcaagatgagcgaggcgttgccgctgggcgccccggacgccggcgctgccctggccggcaagctgaggagcggcgaccgcagcatggtggaggtgctggccgaccacccgggcgagctggtgcgcaccgacagccccaacttcctctgctccgtgctgcctacgcactggcgctgcaacaagaccctgcccatcgctttcaaggtggtggccctaggggatgttccagatggcactctggtcactgtgatggctggcaatgatgaaaactactcggctgagctgagaaatgctaccgcagccatgaagaaccaggttgcaagatttaatgacctcaggtttgtcggtcgaagtggaagagggaaaagcttcactctgaccatcactgtcttcacaaacccaccgcaagtcgccacctaccacagagccatcaaaatcacagtggatgggccccgagaacctcgaagacatcggcagaaactagatgatcagaccaagcccgggagcttgtccttttccgagcggctcagtgaactggagcagctgcggcgcacagccatgagggtcagcccacaccacccagcccccacgcccaaccctcgtgcctccctgaaccactccactgcctttaaccctcagcctcagagtcagatgcaggatacaaggcagatccaaccatccccaccgtggtcctacgatcagtcctaccaatacctgggatccattgcctctccttctgtgcacccagcaacgcccatttcacctggacgtgccagcggcatgacaaccctctctgcagaactttccagtcgactctcaacggcacccgacctgacagcgttcagcgacccgcgccagttccccgcgctgccctccatctccgacccccgcatgcactatccaggcgccttcacctactccccgacgccggtcacctcgggcatcggcatcggcatgtcggccatgggctcggccacgcgctaccacacctacctgccgccgccctaccccggctcgtcgcaagcgcagggaggcccgttccaagccagctcgccctcctaccacctgtactacggcgcctcggccggctcctaccagttctccatggtgggcggcgagcgctcgccgccgcgcatcctgccgccctgcaccaacgcctccaccggctccgcgctgctcaaccccagcctcccgaaccagagcgacgtggtggaggccgagggcagccacagcaactcccccaccaacatggcgccctccgcgcgcctggaggaggccgtgtggaggccctactgaggcgccaggcctggcccggctgggccccgcgggccgccgccttcgcctccgggcgcgcgggcctcctgttcgcgacaagcccgccgggatcccgggccctgggcccggccaccgtcctggggccgagggcgcccgacggccaggatctcgctgtaggtcaggcccgcgcagcctcctgcgcccagaagcccacgccgccgccgtctgctggcgccccggccctcgcggaggtgtccgaggcgacgcacctcgagggtgtccgccggccccagcacccaggggacgcgctggaaagcaaacaggaagattcccggagggaaactgtgaatgcttctgatttagcaatgctgtgaataaaaagaaagattttatacccttgacttaactttttaaccaagttgtttattccaaagagtgtggaattttggttggggtggggggagaggagggatgcaactcgccctgtttggcatctaattcttatttttaatttttccgcaccttatcaattgcaaaatgcgtatttgcatttgggtggtttttatttttatatacgtttatataaatatatataaattgagcttgcttctttcttgctttgaccatggaaagaaatatgattcccttttctttaagttttatttaacttttcttttggacttttgggtagttgtttttttttgttttgttttgtttttttgagaaacagctacagctttgggtcatttttaactactgtattcccacaaggaatccccagatatttatgtatcttgatgttcagacatttatgtgttgataattttttaattatttaaatgtacttatattaagaaaaatatcaagtactacattttcttttgttcttgatagtagccaaagttaaatgtatcacattgaagaaggctagaaaaaaagaatgagtaatgtgatcgcttggttatccagaagtattgtttacattaaactccctttcatgttaatcaaacaagtgagtagctcacgcagcaacgtttttaataggatttttagacactgagggtcactccaaggatcagaagtatggaattttctgccaggctcaacaagggtctcatatctaacttcctccttaaaacagagaaggtcaatctagttccagagggttgaggcaggtgccaataattacatctttggagaggatttgatttctgcccagggatttgctcaccccaaggtcatctgataatttcacagatgctgtgtaacagaacacagccaaagtaaactgtgtaggggagccacatttacataggaaccaaatcaatgaatttaggggttacgattatagcaatttaagggcccaccagaagcaggcctcgaggagtcaatttgcctctgtgtgcctcagtggagacaagtgggaaaacatggtcccacctgtgcgagaccccctgtcctgtgctgctcactcaacaacatctttgtgttgctttcaccaggctgagaccctaccctatggggtatatgggcttttacctgtgcaccagtgtgacaggaaagattcatgtcactactgtccgtggctacaattcaaaggtatccaatgtcgctgtaaattttatggcactatttttattggaggatttggtcagaatgcagttgttgtacaactcataaatactaactgctgattttgacacatgtgtgctccaaatgatctggtggttatttaacgtacctcttaaaattcgttgaaacgatttcaggtcaactctgaagagtatttgaaagcaggacttcagaacagtgtttgatttttattttataaatttaagcattcaaattaggcaaatctttggctgcaggcagcaaaaacagctggacttatttaaaacaacttgtttttgagttttcttatatatatattgattatttgttttacacacatgcagtagcactttggtaagagttaaagagtaaagcagcttatgttgtcaggtcgttcttatctagagaagagctatagcagatctcggacaaactcagaatatattcactttcatttttgacaggattccctccacaactcagtttcatatattattccgtattacatttttgcagctaaattaccataaaatgtcagcaaatgtaaaaatttaatttctgaaaagcaccattagcccatttcccccaaattaaacgtaaatgttttttttcagcacatgttaccatgtctgacctgcaaaaatgctggagaaaaatgaaggaaaaaattatgtttttcagtttaattctgttaactgaagatattccaactcaaaaccagcctcatgctctgattagataatcttttacattgaacctttactctcaaagccatgtgtggagggggcttgtcactattgtaggctcactggattggtcatttagagtttcacagactcttaccagcatatatagtatttaattgtttcaaaaaaaatcaaactgtagttgttttggcgataggtctcacgcaacacatttttgtatgtgtgtgtgtgtgcgtgtgtgtgtgtgtgtgtgaaaaattgcattcattgacttcaggtagattaaggtatctttttattcattgccctcaggaaagttaaggtatcaatgagacccttaagccaatcatgtaataactgcatgtgtctggtccaggagaagtattgaataagccatttctactgcttactcatgtccctatttatgatttcaacatggatacatatttcagttctttctttttctcactatctgaaaatacatttccctccctctcttccccccaatatctccctttttttctctcttcctctatcttccaaaccccactttctccctcctccttttcctgtgttctcttaagcagatagcacatacccccacccagtaccaaatttcagaacacaagaaggtccagttcttcccccttcacataaaggaacatggtttgtcagcctttctcctgtttatgggtttcttccagcagaacagagacattgccaaccatattggatctgcttgctgtccaaaccagcaaactttcctgggcaaatcacaatcagtgagtaaatagacagcctttctgctgccttgggtttctgtgcagataaacagaaatgctctgattagaaaggaaatgaatggttccactcaaatgtcctgcaatttaggattgcagatttctgccttgaaatacctgtttctttgggacattccgtcctgatgatttttatttttgttggtttttatttttggggggaatgacatgtttgggtcttttatacatgaaaatttgtttgacaataatctcacaaaacatattttacatctgaacaaaatgcctttttgtttaccgtagcgtatacatttgttttgggatttttgtgtgtttgttgggaattttgtttttagccaggtcagtattgatgaggctgatcatttggctctttttttccttccagaagagttgcatcaacaaagttaattgtatttatgtatgtaaatagattttaagcttcattataaaatattgttaatgcctataactttttttcaatttttttgtgtgtgtttctaaggactttttcttaggtttgctaaatactgtagggaaaaaaatgcttctttctactttgtttattttagactttaaaatgagctacttcttattcacttttgtaaacagctaatagcatggttccaattttttttaagttcactttttttgttctaggggaaatgaatgtgcaaaaaaagaaaaagaactgttggttatttgtgttattctggatgtataaaaatcaatggaaaaaaataaactttcaaattgaaatgacggtataacacatctactgaaaaagcaacgggaaatgtggtcctatttaagccagcccccacctagggtctatttgtgtggcagttattgggtttggtcacaaaacatcctgaaaattcgtgcgtgggcttctttctccctggtacaaacgtatggaatgcttcttaaaggggaactgtcaagctggtgtcttcagccagatgacatgagagaatatcccagaaccctctctccaaggtgtttctagatagcacaggagagcaggcactgcactgtccacagtccacggtacacagtcgggtgggccgcctcccctctcctgggagcattcgtcgtgcccagcctgagcagggcagctggactgctgctgttcaggagccaccagagccttcctctctttgtaccacagtttcttctgtaaatccagtgttacaatcagtgtgaatggcaaataaacagtttgacaagtacatacaccata

SEQ ID NO: 23 - protein, 326 aa, Homo sapiens
MLLSKFGSLAHLCGPGGVDHLPVKILQPAKADKESFEKAYQVGAVLGSGGFGTVYAGSRIADGLPVAVKHVVKERVTEWGSLGGATVPLEVVLLRKVGAAGGARGVIRLLDWFERPDGFLLVLERPEPAQDLFDFITERGALDEPLARRFFAQVLAAVRHCHSCGVVHRDIKDENLLVDLRSGELKLIDFGSGALLKDTVYTDFDGTRVYSPPEWIRYHRYHGRSATVWSLGVLLYDMVCGDIPFEQDEEILRGRLLFRRRVSPECQQLIRWCLSLRPSERPSLDQIAAHPWMLGADGGVPESCDLRLCTLDPDDVASTTSSSESL

SEQ ID NO: 24 - protein, 326 aa, Homo sapiens
MLLSKFGSLAHLCGPGGVDHLPVKILQPAKADKESFEKAYQVGAVLGSGGFGTVYAGSRIADGLPVAVKHVVKERVTEWGSLGGATVPLEVVLLRKVGAAGGARGVIRLLDWFERPDGFLLVLERPEPAQDLFDFITERGALDEPLARRFFAQVLAAVRHCHSCGVVHRDIKDENLLVDLRSGELKLIDFGSGALLKDTVYTDFDGTRVYSPPEWIRYHRYHGRSATVWSLGVLLYDMVCGDIPFEQDEEILRGRLLFRRRVSPECQQLIRWCLSLRPSERPSLDQIAAHPWMLGADGGAPESCDLRLCTLDPDDVASTTSSSESL

SEQ ID NO: 25 - protein, 326 aa, Homo sapiens; identical to SEQ ID NO: 24

SEQ ID NO: 26 - protein, 326 aa, Homo sapiens
MLLSKFGSLAHLCGPGGVDHLPVKILQPAKADKESFKKAYQVGAVLGSGGFGTVYAGSRIADGLPVAVKHVVKERVTEWGSLGGATVPLEVVLLRKVGAAGGARGVIRLLDWFERPDGFLLVLERPEPAQDLFDFITERGALDEPLARRFFAQVLAAVRHCHSCGVVHRDIKDENLLVDLRSGELKLIDFGSGALLKDTVYTDFDGTRVYSPPEWIRYHRYHGRSATVWSLGVLLYDMVCGDIPFEQDEEILRGRLLFRRRVSPECQQLIRWCLSLRPSERPSLDQIAAHPWMLGADGGAPESCDLRLCTLDPDDVASTTSSSESL

SEQ ID NO: 27 - DNA, 2410 bp, Artificial Sequence
  PIM3 cDNA sequence
gagagcgtgagcgcggagagcggaccgacgcgacacgccgtgcgcctccgcggctgcgctacgaaaacgagtcccggagcggccccgcgcccgccgcacccggccctcgcccgcccgaagacaggcgccaagctgccccgccgtctccccagctagcgcccggccgccgccgcctcgcgggccccgggcggaagggggcggggtcccgattcgccccgcccccgcggagggatacgcggcgccgcggcccaaaacccccgggcgaggcggccggggcgggtgaggcgctccgcctgctgcgcgtctacgcggtccccgcgggccttccgggcccactgcgccgcgcggaccgcctcgggctcggacggccggtgtccccggcgcgccgctcgcccggatcggccgcggcttcggcgcctggggctcggggctccggggaggccgtcgcccgcgatgctgctctccaagttcggctccctggcgcacctctgcgggcccggcggcgtggaccacctcccggtgaagatcctgcagccagccaaggcggacaaggagagcttcgagaaggcgtaccaggtgggcgccgtgctgggtagcggcggcttcggcacggtctacgcgggtagccgcatcgccgacgggctcccggtggctgtgaagcacgtggtgaaggagcgggtgaccgagtggggcagcctgggcggcgcgaccgtgcccctggaggtggtgctgctgcgcaaggtgggcgcggcgggcggcgcgcgcggcgtcatccgcctgctggactggttcgagcggcccgacggcttcctgctggtgctggagcggcccgagccggcgcaggacctcttcgactttatcacggagcgcggcgccctggacgagccgctggcgcgccgcttcttcgcgcaggtgctggccgccgtgcgccactgccacagctgcggggtcgtgcaccgcgacattaaggacgaaaatctgcttgtggacctgcgctccggagagctcaagctcatcgacttcggttcgggtgcgctgctcaaggacacggtctacaccgacttcgacggcacccgagtgtacagccccccggagtggatccgctaccaccgctaccacgggcgctcggccaccgtgtggtcgctgggcgtgcttctctacgatatggtgtgtggggacatccccttcgagcaggacgaggagatcctccgaggccgcctgctcttccggaggagggtctctccagagtgccagcagctgatccggtggtgcctgtccctgcggccctcagagcggccgtcgctggatcagattgcggcccatccctggatgctgggggctgacgggggcgtcccggagagctgtgacctgcggctgtgcaccctcgaccctgatgacgtggccagcaccacgtccagcagcgagagcttgtgaggagctgcacctgactgggagctaggggaccacctgccttggccagacctgggacgcccccagaccctgactttctcctgcgtgggccgtctcctcctgcggaagcagtgacctctgacccctggtgaccttcgctttgagtgccttttgaacgctggtcccgcgggacttggttttctcaagctctgtctgtccaaagacgctccggtcgaggtcccgcctgccctgggtggatacttgaaccccagacgcccctctgtgctgctgtgtccggaggcggccttcccatctgcctgcccacccggagctctttccgccggcgcagggtcccaagcccacctcccgccctcagtcctgcggtgtgcgtctgggcacgtcctgcacacacaatgcaagtcctggcctccgcgcccgcccgcccacgcgagccgtacccgccgccaactctgttatttatggtgtgaccccctggaggtgccctcggcccaccggggctatttattgtttaatttatttgttgaggttatttcctctgagcagtctgcctctcccaagccccaggggacagtggggaggcaggggagggggtggctgtggtccagggaccccaggccctgattcctgtgcctggcgtctgtcccggccccgcctgtcagaagatgaacatgtatagtggctaacttaaggggagtgggtgaccctgacacttccaggcactgtgcccagggtttgggttttaaattattgactttgtacagtctgcttgtgggctctgaaagctggggtggggccagagcctgagcgtttaatttattcagtacctgtgtttgtgtgaatgcggtgtgtgcaggcatcgcagatgggggttctttcagttcaaaagtgagatgtctggagatcatatttttttatacaggtatttcaattaaaatgtttttgtacataaaaaaaaaaaaaaaaaaaaaaaaaaaaaaaa

SEQ ID NO: 28 - DNA, 2004 bp, Artificial Sequence
  PIM3 cDNA sequence
gctcgcccggatcggccgcggcttcggcgcctggggctcggggctccggggaggccgtcgcccgcgatgctgctctccaagttcggctccctggcgcacctctgcgggcccggcggcgtggaccacctcccggtgaagatcctgcagccagccaaggcggacaaggagagcttcaagaaggcgtaccaggtgggcgccgtgctgggtagcggcggcttcggcacggtctacgcgggtagccgcatcgccgacgggctcccggtggctgtgaagcacgtggtgaaggagcgggtgaccgagtggggcagcctgggcggcgcgaccgtgcccctggaggtggtgctgctgcgcaaggtgggcgcggcgggcggcgcgcgcggcgtcatccgcctgctggactggttcgagcggcccgacggcttcctgctggtgctggagcggcccgagccggcgcaggacctcttcgactttatcacggagcgcggcgccctggacgagccgctggcgcgccgcttcttcgcgcaggtgctggccgccgtgcgccactgccacagctgcggggtcgtgcaccgcgacattaaggacgaaaatctgcttgtggacctgcgctccggagagctcaagctcatcgacttcggttcgggtgcgctgctcaaggacacggtctacaccgacttcgacggcacccgagtgtacagccccccggagtggatccgctaccaccgctaccacgggcgctcggccaccgtgtggtcgctgggcgtgcttctctacgatatggtgtgtggggacatccccttcgagcaggacgaggagatcctccgaggccgcctgctcttccggaggagggtctctccagagtgccagcagctgatccggtggtgcctgtccctgcggccctcagagcggccgtcgctggatcagattgcggcccatccctggatgctgggggctgacgggggcgccccggagagctgtgacctgcggctgtgcaccctcgaccctgatgacgtggccagcaccacgtccagcagcgagagcttgtgaggagctgcacctgactgggagctaggggaccacctgccttggccagacctgggacgcccccagaccctgactttttcctgcgtgggccgtctcctcctgcggaagcagtgacctctgacccctggtgaccttcgctttgagtgccttttgaacgctggtcccgcgggacttggttttctcaagctctgtctgtccaaagaggctccagtcgaggtcccgcctgccctgggtggatacttgaaccccagacgcccctctgtgctgctgtgtccggaggcggccttcccatctgcctgcccacccggagctctttccgccggcgcagggtcccaagcccacctcccgccctcagtcctgcggtgtgcgtctgggcacgtcctgcacacacaatgcaagtcctggcctccgcgcccgcccgcccacgcgagccgtacccgccgccaactctgttatttatggtgtgaccccctggaggtgccctcggcccaccggggctatttattgtttaatttatttgttgaggttatttcctctgagcagtctgcctctcccaagccccaggggacagtggggggcaggggagggggtggctttggtccagggaccccaggccctgattcctgtgcctggcgtctgtcctggccccgcctgtcagaagatgaacatgtgtagtggctaacttaaggggagtgggtgaccctgacacttccaggcactgtgcccagggtttgggttttaaattattgactttgtacagtctgcttgtgggctctgaaagctggggtggggccagagcctgagcgtttaatttattcagtacctgtgtttgtgtgaatgcggtgtgtgcaggcatcgcagatgggggttctttcagttcaaaagtgagatgtctggagatcatatttttttatacaggtatttcaattaaaatgtttttgtacaaaaaaaaaaaaaaaa

SEQ ID NO: 29 - DNA, 2392 bp, Artificial Sequence
  PIM3 cDNA sequence
agcggaccgacgcgacacgccgtgcgcctccgcggctgcgctacgaaaacgagtcccggagcggccccgcgcccgccgcacccggccctcgcccacccgaagacaggcgcccagctgccccgccgtctccccagctagcgcccggccgccgccgcctcgcgggccccgggcggaagggggcggggtcccgattcgccccgcccccgcggagggatacgcggcgccgcggcccaaaacccccgggcgaggcggccggggcgggtgaggcgctccgcctgctgctcgtctacgcggtccccgcgggccttccgggcccactgcgccgcgcggaccgcctcgggctcggacggccggtgtccccggcgcgccgctcgcccggatcggccgcggcttcggcgcctggggctcggggctccggggaggccgtcgcccgcgatgctgctctccaagttcggctccctggcgcacctctgcgggcccggcggcgtggaccacctcccggtgaagatcctgcagccagccaaggcggacaaggagagcttcgagaaggcgtaccaggtgggcgccgtgctgggtagcggcggcttcggcacggtctacgcgggtagccgcatcgccgacgggctcccggtggctgtgaagcacgtggtgaaggagcgggtgaccgagtggggcagcctgggcggcgcgaccgtgcccctggaggtggtgctgctgcgcaaggtgggcgcggcgggcggcgcgcgcggcgtcatccgcctgctggactggttcgagcggcccgacggcttcctgctggtgctggagcggcccgagccggcgcaggacctcttcgactttatcacggagcgcggcgccctggacgagccgctggcgcgccgcttcttcgcgcaggtgctggccgccgtgcgccactgccacagctgcggggtcgtgcaccgcgacattaaggacgaaaatctgcttgtggacctgcgctccggagagctcaagctcatcgacttcggttcgggtgcgctgctcaaggacacggtctacaccgacttcgacggcacccgagtgtacagccccccggagtggatccgctaccaccgctaccacgggcgctcggccaccgtgtggtcgctgggcgtgcttctctacgatatggtgtgtggggacatccccttcgagcaggacgaggagatcctccgaggccgcctgctcttccggaggagggtctctccagagtgccagcagctgatccggtggtgcctgtccctgcggccctcagagcggccgtcgctggatcagattgcggcccatccctggatgctgggggctgacgggggcgccccggagagctgtgacctgcggctgtgcaccctcgaccctgatgacgtggccagcaccacgtccagcagcgagagcttgtgaggagctgcacctgactgggagctaggggaccacctgccttggccagacctgggacgcccccagaccctgactttttcctgcgtgggccgtctcctcctgcggaagcagtgacctctgacccctggtgaccttcgctttgagtgccttttgaacgctggtcccgcgggacttggttttctcaagctctgtctgtccaaagacgctccggtcgaggtcccgcctgccctgggtggatacttgaaccccagacgcccctctgtgctgctgtgtccggaggcggccttcccatctgcctgcccacccggagctctttccgccggcgcagggtcccaagcccacctcccgccctcagtcctgcggtgtgcgtctgggcacgtcctgcacacacaatgcaagtcctggcctccgcgcccgcccgcccacgcgagccgtacccgccgccaactctgttatttatggtgtgaccccctggaggtgccctcggcccaccggggctatttattgtttaatttatttgttgaggttatttcctctgagcagtctgcctctcccaagccccaggggacagtggggaggcaggggagggggtggctgtggtccagggaccccaggccctgattcctgtgcctggcgtctgtcctggccccgcctgtcagaagatgaacatgtatagtggctaacttaaggggagtgggtgaccctgacacttccaggcactgtgcccagggtttgggttttaaattattgactttgtacagtctgcttgtgggctctgaaagctggggtggggccagagcctgagcgtttaatttattcagtacctgtgtttgtgtgaatgcggtgtgtgcaggcatcgcagatgggggttctttcagttcaaaagtgagatgtctggagatcatatttttttatacaggtatttcaattaaaatgtttttgtacataaaaaaaaaaaaaaaaaaaaaaaaaaaaaaaa

SEQ ID NO: 30 - DNA, 1524 bp, Artificial Sequence
  PIM3 cDNA sequence
tctcgggctcggacggccggtgtccccggcgcgccgctcgcccggatcggccgcggcttcggcgcctggggctcggggctccggggaggccgtcgcccgcgatgctgctctccaagttcggctccctggcgcacctctgcgggcccggcggcgtggaccacctcccggtgaagatcctgcagccagccaaggcggacaaggagagcttcgagaaggcgtaccaggtgggcgccgtgctgggtagcggcggcttcggcacggtctacgcgggtagccgcatcgccgacgggctcccggtggctgtgaagcacgtggtgaaggagcgggtgaccgagtggggcagcctgggcggcgcgaccgtgcccctggaggtggtgctgctgcgcaaggtgggcgcggcgggcggcgcgcgcggcgtcatccgcctgctggactggttcgagcggcccgacggcttcctgctggtgctggagcggcccgagccggcgcaggacctcttcgactttatcacggagcgcggcgccctggacgagccgctggcgcgccgcttcttcgcgcaggtgctggccgccgtgcgccactgccacagctgcggggtcgtgcaccgcgacattaaggacgaaaatctgcttgtggacctgcgctccggagagctcaagctcatcgacttcggttcgggtgcgctgctcaaggacacggtctacaccgacttcgacggcacccgagtgtacagccccccggagtggatccgctaccaccgctaccacgggcgctcggccaccgtgtggtcgctgggcgtgcttctctacgatatggtgtgtggggacatccccttcgagcaggacgaggagatcctccgaggccgcctgctcttccggaggagggtctctccagagtgccagcagctgatccggtggtgcctgtccctgcggccctcagagcggccgtcgctggatcagattgcggcccatccctggatgctgggggctgacgggggcgccccggagagctgtgacctgcggctgtgcaccctcgaccctgatgacgtggccagcaccacgtccagcagcgagagcttgtgaggagctgcacctgactgggagctaggggaccacctgccttggccagacctgggacgcccccagaccctgaccttttcctgcgtgggccgtctcctcctgcggaagcagtgacctctgacccctggtgaccttcgctttgagtgccttttgaacgctggtcccgcgggacttggttttctcaagctctgtctgtccaaagacgctccggtcgaggtcccgcctgccctgggtggatacttgaaccccagacgcccctctgtgctgctgtgtccggaggcggccttcccatctgcctgcccacccggagctctttccgccggcgcagggtcccaagcccacctcccgccctcagtcctgcggtgtgcgtctgggcacgtcctgcacacacaatgcaagtcctggcctccgcgcccgcccgcccacgcgagccgtacccgccgcc

SEQ ID NO: 31 - protein, 291 aa, Homo sapiens
MQRARPTLWAAALTLLVLLRGPPVARAGASSAGLGPVVRCEPCDARALAQCAPPPAVCAELVREPGCGCCLTCALSEGQPCGIYTERCGSGLRCQPSPDEARPLQALLDGRGLCVNASAVSRLRAYLLPAPPAPGNASESEEDRSAGSVESPSVSSTHRVSDPKFHPLHSKIIIIKKGHAKDSQRYKVDYESQSTDTQNFSSESKRETEYGPCRREMEDTLNHLKFLNVLSPRGVHIPNCDKKGFYKKKQCRPSKGRKRGFCWCVDKYGQPLPGYTTKGKEDVHCYSMQSK

SEQ ID NO: 32 - protein, 297 aa, Homo sapiens
MQRARPTLWAAALTLLVLLRGPPVARAGASSAGLGPVVRCEPCDARALAQCAPPPAVCAELVREPGCGCCLTCALSEGQPCGIYTERCGSGLRCQPSPDEARPLQALLDGRGLCVNASAVSRLRAYLLPAPPAPGEPPAPGNASESEEDRSAGSVESPSVSSTHRVSDPKFHPLHSKIIIIKKGHAKDSQRYKVDYESQSTDTQNFSSESKRETEYGPCRREMEDTLNHLKFLNVLSPRGVHIPNCDKKGFYKKKQCRPSKGRKRGFCWCVDKYGQPLPGYTTKGKEDVHCYSMQSK

SEQ ID NO: 33 - protein, 291 aa, homo sapiens; identical to SEQ ID NO: 31

SEQ ID NO: 34 - protein, 297 aa, homo sapiens; identical to SEQ ID NO: 32

SEQ ID NO: 35 - DNA, 2638 bp, Artificial Sequence
  IGFBP3 cDNA sequence
agatgcgagcactgcggctgggcgctgaggatcagccgcttcctgcctggattccacagcttcgcgccgtgtactgtcgccccatccctgcgcgcccagcctgccaagcagcgtgccccggttgcaggcgtcatgcagcgggcgcgacccacgctctgggccgctgcgctgactctgctggtgctgctccgcgggccgccggtggcgcgggctggcgcgagctcggcgggcttgggtcccgtggtgcgctgcgagccgtgcgacgcgcgtgcactggcccagtgcgcgcctccgcccgccgtgtgcgcggagctggtgcgcgagccgggctgcggctgctgcctgacgtgcgcactgagcgagggccagccgtgcggcatctacaccgagcgctgtggctccggccttcgctgccagccgtcgcccgacgaggcgcgaccgctgcaggcgctgctggacggccgcgggctctgcgtcaacgctagtgccgtcagccgcctgcgcgcctacctgctgccagcgccgccagctccaggtgagccgcccgcgccaggaaatgctagtgagtcggaggaagaccgcagcgccggcagtgtggagagcccgtccgtctccagcacgcaccgggtgtctgatcccaagttccaccccctccattcaaagataatcatcatcaagaaagggcatgctaaagacagccagcgctacaaagttgactacgagtctcagagcacagatacccagaacttctcctccgagtccaagcgggagacagaatatggtccctgccgtagagaaatggaagacacactgaatcacctgaagttcctcaatgtgctgagtcccaggggtgtacacattcccaactgtgacaagaagggattttataagaaaaagcagtgtcgcccttccaaaggcaggaagcggggcttctgctggtgtgtggataagtatgggcagcctctcccaggctacaccaccaaggggaaggaggacgtgcactgctacagcatgcagagcaagtagacgcctgccgcaaggttaatgtggagctcaaatatgccttattttgcacaaaagactgccaaggacatgaccagcagctggctacagcctcgatttatatttctgtttgtggtgaactgattttttttaaaccaaagtttagaaagaggtttttgaaatgcctatggtttctttgaatggtaaacttgagcatcttttcactttccagtagtcagcaaagagcagtttgaattttcttgtcgcttcctatcaaaatattcagagactcgagcacagcacccagacttcatgcgcccgtggaatgctcaccacatgttggtcgaagcggccgaccactgactttgtgacttaggcggctgtgttgcctatgtagagaacacgcttcacccccactccccgtacagtgcgcacaggctttatcgagaataggaaaacctttaaaccccggtcatccggacatcccaacgcatgctcctggagctcacagccttctgtggtgtcatttctgaaacaagggcgtggatccctcaaccaagaagaatgtttatgtcttcaagtgacctgtactgcttggggactattggagaaaataaggtggagtcctacttgtttaaaaaatatgtatctaagaatgttctagggcactctgggaacctataaaggcaggtatttcgggccctcctcttcaggaatcttcctgaagacatggcccagtcgaaggcccaggatggcttttgctgcggccccgtggggtaggagggacagagagacagggagagtcagcctccacattcagaggcatcacaagtaatggcacaattcttcggatgactgcagaaaatagtgttttgtagttcaacaactcaagacgaagcttatttctgaggataagctctttaaaggcaaagctttattttcatctctcatcttttgtcctccttagcacaatgtaaaaaagaatagtaatatcagaacaggaaggaggaatggcttgctggggagcccatccaggacactgggagcacatagagattcacccatgtttgttgaacttagagtcattctcatgcttttctttataattcacacatatatgcagagaagatatgttcttgttaacattgtatacaacatagccccaaatatagtaagatctatactagataatcctagatgaaatgttagagatgctatatgatacaactgtggccatgactgaggaaaggagctcacgcccagagactgggctgctctcccggaggccaaacccaagaaggtctggcaaagtcaggctcagggagactctgccctgctgcagacctcggtgtggacacacgctgcatagagctctccttgaaaacagaggggtctcaagacattctgcctacctattagcttttctttatttttttaactttttggggggaaaagtatttttgagaagtttgtcttgcaatgtatttataaatagtaaataaagtttttaccattaaaaaaatatctttccctttgttattgaccatctctgggctttgtatcactaattattttattttattatataataattattttattataataaaatcctgaaaggggaaaataaaaaaaa

SEQ ID NO: 36 - DNA, 2620 bp, Artificial Sequence
  IGFBP3 cDNA sequence
agatgcgagcactgcggctgggcgctgaggatcagccgcttcctgcctggattccacagcttcgcgccgtgtactgtcgccccatccctgcgcgcccagcctgccaagcagcgtgccccggttgcaggcgtcatgcagcgggcgcgacccacgctctgggccgctgcgctgactctgctggtgctgctccgcgggccgccggtggcgcgggctggcgcgagctcggcgggcttgggtcccgtggtgcgctgcgagccgtgcgacgcgcgtgcactggcccagtgcgcgcctccgcccgccgtgtgcgcggagctggtgcgcgagccgggctgcggctgctgcctgacgtgcgcactgagcgagggccagccgtgcggcatctacaccgagcgctgtggctccggccttcgctgccagccgtcgcccgacgaggcgcgaccgctgcaggcgctgctggacggccgcgggctctgcgtcaacgctagtgccgtcagccgcctgcgcgcctacctgctgccagcgccgccagctccaggaaatgctagtgagtcggaggaagaccgcagcgccggcagtgtggagagcccgtccgtctccagcacgcaccgggtgtctgatcccaagttccaccccctccattcaaagataatcatcatcaagaaagggcatgctaaagacagccagcgctacaaagttgactacgagtctcagagcacagatacccagaacttctcctccgagtccaagcgggagacagaatatggtccctgccgtagagaaatggaagacacactgaatcacctgaagttcctcaatgtgctgagtcccaggggtgtacacattcccaactgtgacaagaagggattttataagaaaaagcagtgtcgcccttccaaaggcaggaagcggggcttctgctggtgtgtggataagtatgggcagcctctcccaggctacaccaccaaggggaaggaggacgtgcactgctacagcatgcagagcaagtagacgcctgccgcaaggttaatgtggagctcaaatatgccttattttgcacaaaagactgccaaggacatgaccagcagctggctacagcctcgatttatatttctgtttgtggtgaactgattttttttaaaccaaagtttagaaagaggtttttgaaatgcctatggtttctttgaatggtaaacttgagcatcttttcactttccagtagtcagcaaagagcagtttgaattttcttgtcgcttcctatcaaaatattcagagactcgagcacagcacccagacttcatgcgcccgtggaatgctcaccacatgttggtcgaagcggccgaccactgactttgtgacttaggcggctgtgttgcctatgtagagaacacgcttcacccccactccccgtacagtgcgcacaggctttatcgagaataggaaaacctttaaaccccggtcatccggacatcccaacgcatgctcctggagctcacagccttctgtggtgtcatttctgaaacaagggcgtggatccctcaaccaagaagaatgtttatgtcttcaagtgacctgtactgcttggggactattggagaaaataaggtggagtcctacttgtttaaaaaatatgtatctaagaatgttctagggcactctgggaacctataaaggcaggtatttcgggccctcctcttcaggaatcttcctgaagacatggcccagtcgaaggcccaggatggcttttgctgcggccccgtggggtaggagggacagagagacagggagagtcagcctccacattcagaggcatcacaagtaatggcacaattcttcggatgactgcagaaaatagtgttttgtagttcaacaactcaagacgaagcttatttctgaggataagctctttaaaggcaaagctttattttcatctctcatcttttgtcctccttagcacaatgtaaaaaagaatagtaatatcagaacaggaaggaggaatggcttgctggggagcccatccaggacactgggagcacatagagattcacccatgtttgttgaacttagagtcattctcatgcttttctttataattcacacatatatgcagagaagatatgttcttgttaacattgtatacaacatagccccaaatatagtaagatctatactagataatcctagatgaaatgttagagatgctatatgatacaactgtggccatgactgaggaaaggagctcacgcccagagactgggctgctctcccggaggccaaacccaagaaggtctggcaaagtcaggctcagggagactctgccctgctgcagacctcggtgtggacacacgctgcatagagctctccttgaaaacagaggggtctcaagacattctgcctacctattagcttttctttatttttttaactttttggggggaaaagtatttttgagaagtttgtcttgcaatgtatttataaatagtaaataaagtttttaccattaaaaaaatatctttccctttgttattgaccatctctgggctttgtatcactaattattttattttattatataataattattttattataataaaatcctgaaaggggaaaataaaaaaaa

SEQ ID NO: 37 - DNA, 20 bp, Artificial Sequence
  AIF1 Forward Primer Sequence
gatgatgctgggcaagagat

SEQ ID NO: 38 - DNA, 20 bp, Artificial Sequence
  AIF1 Reverse primer Sequence
ccttcaaatcagggcaactc

SEQ ID NO: 39 - DNA, 20 bp, Artificial Sequence
  AMPD3 Forward Primer Sequence
aaaaggaagccaaggagagg

SEQ ID NO: 40 - DNA, 20 bp, Artificial Sequence
  AMPD3 Reverse primer Sequence
gggaccgaatcatcttgaaa

SEQ ID NO: 41 - DNA, 20 bp, Artificial Sequence
  APOE Forward Primer Sequence
ttctgtgggctgcgttgctg

SEQ ID NO: 42 - DNA, 20 bp, Artificial Sequence
  APOE Reverse primer Sequence
tacactgccaggcgcttctg

SEQ ID NO: 43 - DNA, 21 bp, Artificial Sequence
  ARL4C Forward Primer Sequence
ccagtccctgcatatcgtcat

SEQ ID NO: 44 - DNA, 22 bp, Artificial Sequence
  ARL4C Reverse primer Sequence
ttcacgaactcgttgaacttga

SEQ ID NO: 45 - DNA, 23 bp, Artificial Sequence
  ATP6AP2 Forward Primer Sequence
agggagtgaacaaactggctcta

SEQ ID NO: 46 - DNA, 30 bp, Artificial Sequence
  ATP6AP2 Reverse primer Sequence
taccatatacactctattctccaaagggta

SEQ ID NO: 47 - DNA, 19 bp, Artificial Sequence
  AXL Forward Primer Sequence
ccgtggacctactctggct

SEQ ID NO: 48 - DNA, 19 bp, Artificial Sequence
  AXL Reverse primer Sequence
ccttggcgttatgggcttc

SEQ ID NO: 49 - DNA, 20 bp, Artificial Sequence
  B2M Forward Primer Sequence
actgaattcacccccactga

SEQ ID NO: 50 - DNA, 20 bp, Artificial Sequence
  B2M Reverse primer Sequence
cctccatgatgctgcttaca

SEQ ID NO: 51 - DNA, 20 bp, Artificial Sequence
  BASP1 Forward Primer Sequence
cggagcccacttagcttgtc

SEQ ID NO: 52 - DNA, 24 bp, Artificial Sequence
  BASP1 Reverse primer Sequence
gagagaatgtttgtcactcccaaa

SEQ ID NO: 53 - DNA, 20 bp, Artificial Sequence
  BGN Forward Primer Sequence
ctggcatccccaaagacctc

SEQ ID NO: 54 - DNA, 20 bp, Artificial Sequence
  BGN Reverse primer Sequence
gctcccgttctcgatcatcc

SEQ ID NO: 55 - DNA, 20 bp, Artificial Sequence
  BMF Forward Primer Sequence
gacccaacccgggagcttgc

SEQ ID NO: 56 - DNA, 20 bp, Artificial Sequence
  BMF Reverse primer Sequence
gaaggccagggccacagcag

SEQ ID NO: 57 - DNA, 19 bp, Artificial Sequence
  C10orf10 Forward Primer Sequence
tgcccacaattcgggagac

SEQ ID NO: 58 - DNA, 21 bp, Artificial Sequence
  C10orf10 Reverse primer Sequence
agacctcacgtagtcatccag

SEQ ID NO: 59 - DNA, 20 bp, Artificial Sequence
  CCL2 Forward Primer Sequence
gcctccagcatgaaagtctc

SEQ ID NO: 60 - DNA, 19 bp, Artificial Sequence
  CCL2 Reverse primer Sequence
aggtgactggggcattgat

SEQ ID NO: 61 - DNA, 20 bp, Artificial Sequence
  CCL20 Forward Primer Sequence
gtgctgctactccacctctg

SEQ ID NO: 62 - DNA, 20 bp, Artificial Sequence
  CCL20 Reverse primer Sequence
cgtgtgaagcccacaataaa

SEQ ID NO: 63 - DNA, 20 bp, Artificial Sequence
  CCND1 Forward Primer Sequence
gctgcgaagtggaaaccatc

SEQ ID NO: 64 - DNA, 22 bp, Artificial Sequence
  CCND1 Reverse primer Sequence
cctccttctgcacacatttgaa

SEQ ID NO: 65 - DNA, 19 bp, Artificial Sequence
  CD14 Forward Primer Sequence
acgccagaaccttgtgagc

SEQ ID NO: 66 - DNA, 22 bp, Artificial Sequence
  CD14 Reverse primer Sequence
gcatggatctccacctctactg

SEQ ID NO: 67 - DNA, 21 bp, Artificial Sequence
  CD300LF Forward Primer Sequence
ggaaccgacctactgcaacat

SEQ ID NO: 68 - DNA, 21 bp, Artificial Sequence
  CD300LF Reverse primer Sequence
ctgatggtgctgtattccgtg

SEQ ID NO: 69 - DNA, 20 bp, Artificial Sequence
  CD44 Forward Primer Sequence
cggacaccatggacaagttt

SEQ ID NO: 70 - DNA, 20 bp, Artificial Sequence
  CD44 Reverse primer Sequence
gaaagccttgcagaggtcag

SEQ ID NO: 71 - DNA, 20 bp, Artificial Sequence
  CD83 Forward Primer Sequence
ctccgaagatgtggacttgc

SEQ ID NO: 72 - DNA, 20 bp, Artificial Sequence
  CD83 Reverse primer Sequence
tccatcctctcttcaccacc

SEQ ID NO: 73 - DNA, 20 bp, Artificial Sequence
  CDCP1 Forward Primer Sequence
ctgaactgcggggtctctat

SEQ ID NO: 74 - DNA, 20 bp, Artificial Sequence
  CDCP1 Reverse primer Sequence
ggcagagcaatctcaaaagc

SEQ ID NO: 75 - DNA, 23 bp, Artificial Sequence
  CDH13 Forward Primer Sequence
agtgttccatatcaatcagccag

SEQ ID NO: 76 - DNA, 21 bp, Artificial Sequence
  CDH13 Reverse primer Sequence
cgagacctcatagcgtagctt

SEQ ID NO: 77 - DNA, 20 bp, Artificial Sequence
  CECR1 Forward Primer Sequence
cagagagcatctggcttcaa

SEQ ID NO: 78 - DNA, 20 bp, Artificial Sequence
  CECR1 Reverse primer Sequence
tcatggtgctctccactgag

SEQ ID NO: 79 - DNA, 22 bp, Artificial Sequence
  CHMP1B Forward Primer Sequence
aaagaactgagtaggagtgcca

SEQ ID NO: 80 - DNA, 22 bp, Artificial Sequence
  CHMP1B Reverse primer Sequence
tgtatcctcgcaacttccatgt

SEQ ID NO: 81 - DNA, 20 bp, Artificial Sequence
  CHST11 Forward Primer Sequence
tccctttggtgtggacatct

SEQ ID NO: 82 - DNA, 20 bp, Artificial Sequence
  CHST11 Reverse primer Sequence
gcaggacagcagtgtttgag

SEQ ID NO: 83 - DNA, 20 bp, Artificial Sequence
  COLEC12 Forward Primer Sequence
agaggaggaggaggtgcaat

SEQ ID NO: 84 - DNA, 22 bp, Artificial Sequence
  COLEC12 Reverse primer Sequence
tgatagaaaacttcagtgccca

SEQ ID NO: 85 - DNA, 21 bp, Artificial Sequence
  CREG1 Forward Primer Sequence
ggcgtgccctatttctacctg

SEQ ID NO: 86 - DNA, 23 bp, Artificial Sequence
  CREG1 Reverse primer Sequence
caaagtcatggtcagtgtagcat

SEQ ID NO: 87 - DNA, 20 bp, Artificial Sequence
  CST3 Forward Primer Sequence
ccagcaacgacatgtaccac

SEQ ID NO: 88 - DNA, 20 bp, Artificial Sequence
  CST3 Reverse primer Sequence
cagctccacgtccaagaagt

SEQ ID NO: 89 - DNA, 21 bp, Artificial Sequence
  CTSB Forward Primer Sequence
acaacgtggacatgagctact

SEQ ID NO: 90 - DNA, 23 bp, Artificial Sequence
  CTSB Reverse primer Sequence
tcggtaaacataactctctgggg

SEQ ID NO: 91 - DNA, 17 bp, Artificial Sequence
  CTSD Forward Primer Sequence
agccctccagccttctg

SEQ ID NO: 92 - DNA, 19 bp, Artificial Sequence
  CTSD Reverse primer Sequence
cggatggacgtgaacttgt

SEQ ID NO: 93 - DNA, 17 bp, Artificial Sequence
  CTSL Forward Primer Sequence
gcgcgtgactggttgag

SEQ ID NO: 94 - DNA, 20 bp, Artificial Sequence
  CTSL Reverse primer Sequence
aaaggcagcaaggatgagtg

SEQ ID NO: 95 - DNA, 21 bp, Artificial Sequence
  CTSS Forward Primer Sequence
cttgtggttggctatggtgat

SEQ ID NO: 96 - DNA, 20 bp, Artificial Sequence
  CTSS Reverse primer Sequence
cctttatttcttgccatccg

SEQ ID NO: 97 - DNA, 19 bp, Artificial Sequence
  CXCL16 Forward Primer Sequence
gtgtgtggaggcaacaagg

SEQ ID NO: 98 - DNA, 20 bp, Artificial Sequence
  CXCL16 Reverse primer Sequence
cacaatccccgagtaagcat

SEQ ID NO: 99 - DNA, 20 bp, Artificial Sequence
  CXCL2 Forward Primer Sequence
gggcagaaagcttgtctcaa

SEQ ID NO: 100 - DNA, 20 bp, Artificial Sequence
  CXCL2 Reverse primer Sequence
gcttcctccttccttctggt

SEQ ID NO: 101 - DNA, 18 bp, Artificial Sequence
  CXCR4 Forward Primer Sequence
ccagtagccaccgcatct

SEQ ID NO: 102 - DNA, 20 bp, Artificial Sequence
  CXCR4 Reverse primer Sequence
atagtcccctgagcccattt

SEQ ID NO: 103 - DNA, 20 bp, Artificial Sequence
  DBI Forward Primer Sequence
tggccactacaaacaagcaa

SEQ ID NO: 104 - DNA, 20 bp, Artificial Sequence
  DBI Reverse primer Sequence
tccctttcagctcattccag

SEQ ID NO: 105 - DNA, 19 bp, Artificial Sequence
  DHRS3 Forward Primer Sequence
ttcctgccacgtatgctgg

SEQ ID NO: 106 - DNA, 22 bp, Artificial Sequence
  DHRS3 Reverse primer Sequence
tttggatgtgcagtagtcgatg

SEQ ID NO: 107 - DNA, 20 bp, Artificial Sequence
  EGR2 Forward Primer Sequence
ttgaccagatgaacggagtg

SEQ ID NO: 108 - DNA, 20 bp, Artificial Sequence
  EGR2 Reverse primer Sequence
agcaaagctgctgggatatg

SEQ ID NO: 109 - DNA, 17 bp, Artificial Sequence
  EPB41L3 Forward Primer Sequence
gagcctagtccccacgc

SEQ ID NO: 110 - DNA, 20 bp, Artificial Sequence
  EPB41L3 Reverse primer Sequence
gcttggattccgagtctgat

SEQ ID NO: 111 - DNA, 22 bp, Artificial Sequence
  EZR Forward Primer Sequence
accaatcaatgtccgagttacc

SEQ ID NO: 112 - DNA, 22 bp, Artificial Sequence
  EZR Reverse primer Sequence
gccgatagtctttaccacctga

SEQ ID NO: 113 - DNA, 20 bp, Artificial Sequence
  FAM49A Forward Primer Sequence
agctaagctggttcatccca

SEQ ID NO: 114 - DNA, 20 bp, Artificial Sequence
  FAM49A Reverse primer Sequence
gactttgagcaggtttccca

SEQ ID NO: 115 - DNA, 22 bp, Artificial Sequence
  FAT1 Forward Primer Sequence
catcctgtcaagatgggtgttt

SEQ ID NO: 116 - DNA, 23 bp, Artificial Sequence
  FAT1 Reverse primer Sequence
tccgagaatgtactcttcagctt

SEQ ID NO: 117 - DNA, 20 bp, Artificial Sequence
  FSCN1 Forward Primer Sequence
caaggacgagctctttgctc

SEQ ID NO: 118 - DNA, 20 bp, Artificial Sequence
  FSCN1 Reverse primer Sequence
tgattggcagacaggtccat

SEQ ID NO: 119 - DNA, 17 bp, Artificial Sequence
  G0S2 Forward Primer Sequence
ctgaccgctgccaactg

SEQ ID NO: 120 - DNA, 20 bp, Artificial Sequence
  G0S2 Reverse primer Sequence
ctcctggaccgtttccatct

SEQ ID NO: 121 - DNA, 20 bp, Artificial Sequence
  GAL3ST4 Forward Primer Sequence
tccacatcctctgtcaccac

SEQ ID NO: 122 - DNA, 20 bp, Artificial Sequence
  GAL3ST4 Reverse primer Sequence
ggtctcggacaatggaaaaa

SEQ ID NO: 123 - DNA, 21 bp, Artificial Sequence
  GPR183 Forward Primer Sequence
actggagaatcggagatgcct

SEQ ID NO: 124 - DNA, 22 bp, Artificial Sequence
  GPR183 Reverse primer Sequence
aatgaagcggtcaatactcagg

SEQ ID NO: 125 - DNA, 20 bp, Artificial Sequence
  GPX1 Forward Primer Sequence
caaccagtttgggcatcagr

SEQ ID NO: 126 - DNA, 19 bp, Artificial Sequence
  GPX1 Reverse primer Sequence
gttcacctcgcacttctcg

SEQ ID NO: 127 - DNA, 19 bp, Artificial Sequence
  GRN Forward Primer Sequence
aggagaacgctaccacgga

SEQ ID NO: 128 - DNA, 21 bp, Artificial Sequence
  GRN Reverse primer Sequence
ggcagcaggtatagccatctg

SEQ ID NO: 129 - DNA, 20 bp, Artificial Sequence
  GTF2B Forward Primer Sequence
gccggtgatatgatctgtcc

SEQ ID NO: 130 - DNA, 20 bp, Artificial Sequence
  GTF2B Reverse primer Sequence
gtcattgctgaaagttcgcc

SEQ ID NO: 131 - DNA, 20 bp, Artificial Sequence
  HES1 Forward Primer Sequence
acgtgcgagggcgttaatac

SEQ ID NO: 132 - DNA, 20 bp, Artificial Sequence
  HES1 Reverse primer Sequence
ggggtaggtcatggcattga

SEQ ID NO: 133 - DNA, 20 bp, Artificial Sequence
  HIF3A Forward Primer Sequence
cccagtcggagagtatcgtc

SEQ ID NO: 134 - DNA, 20 bp, Artificial Sequence
  HIF3A Reverse primer Sequence
gaatgggtctgcgagagtgt

SEQ ID NO: 135 - DNA, 21 bp, Artificial Sequence
  HPRT1 Forward Primer Sequence
cctggcgtcgtgattagtgat

SEQ ID NO: 136 - DNA, 22 bp, Artificial Sequence
  HPRT1 Reverse primer Sequence
agacgttcagtcctgtccataa

SEQ ID NO: 137 - DNA, 20 bp, Artificial Sequence
  HTRA1 Forward Primer Sequence
tggaatctcctttgcaatcc

SEQ ID NO: 138 - DNA, 20 bp, Artificial Sequence
  HTRA1 Reverse primer Sequence
ttcttggtgatggcttttcc

SEQ ID NO: 139 - DNA, 20 bp, Artificial Sequence
  IDH1 Forward Primer Sequence
gtcgtcatgcttatggggat

SEQ ID NO: 140 - DNA, 20 bp, Artificial Sequence
  IDH1 Reverse primer Sequence
cttttgggttccgtcacttg

SEQ ID NO: 141 - DNA, 20 bp, Artificial Sequence
  IFI30 Forward Primer Sequence
gctagccttcctgaccattg

SEQ ID NO: 142 - DNA, 20 bp, Artificial Sequence
  IFI30 Reverse primer Sequence
ccatgatagtgtctggcgac

SEQ ID NO: 143 - DNA, 20 bp, Artificial Sequence
  IGFBP3 Forward Primer Sequence
ctctgcgtcaacgctagtgc

SEQ ID NO: 144 - DNA, 20 bp, Artificial Sequence
  IGFBP3 Reverse primer Sequence
cggtcttcctccgactcact

SEQ ID NO: 145 - DNA, 21 bp, Artificial Sequence
  IRAK2 Forward Primer Sequence
ctgccaccccaatgtcttacc

SEQ ID NO: 146 - DNA, 21 bp, Artificial Sequence
  IRAK2 Reverse primer Sequence
agggaaccatttgccatgtag

SEQ ID NO: 147 - DNA, 20 bp, Artificial Sequence
  IRS2 Forward Primer Sequence
acctacgccagcattgactt

SEQ ID NO: 148 - DNA, 21 bp, Artificial Sequence
  IRS2 Reverse primer Sequence
catcctggtgataaagccaga

SEQ ID NO: 149 - DNA, 20 bp, Artificial Sequence
  LAPTM5 Forward Primer Sequence
agacctgctgctgcttcaat

SEQ ID NO: 150 - DNA, 20 bp, Artificial Sequence
  LAPTM5 Reverse primer Sequence
catgggccacctctactgag

SEQ ID NO: 151 - DNA, 20 bp, Artificial Sequence
  LGALS1 Forward Primer Sequence
tcgccagcaacctgaatctc

SEQ ID NO: 152 - DNA, 20 bp, Artificial Sequence
  LGALS1 Reverse primer Sequence
gcacgaagctcttagcgtca

SEQ ID NO: 153 - DNA, 17 bp, Artificial Sequence
  LGALS3BP Forward Primer Sequence
gaggaggctccacacgg

SEQ ID NO: 154 - DNA, 18 bp, Artificial Sequence
  LGALS3BP Reverse primer Sequence
agcagccacacccagaag

SEQ ID NO: 155 - DNA, 20 bp, Artificial Sequence
  LGMN Forward Primer Sequence
ctgaagatggaggcaagcac

SEQ ID NO: 156 - DNA, 20 bp, Artificial Sequence
  LGMN Reverse primer Sequence
ttgcggtgaatgatctggta

SEQ ID NO: 157 - DNA, 20 bp, Artificial Sequence
  LHFPL2 Forward Primer Sequence
tcttcaatgtctgtgggctg

SEQ ID NO: 158 - DNA, 20 bp, Artificial Sequence
  LHFPL2 Reverse primer Sequence
gtctatggccttctggcaac

SEQ ID NO: 159 - DNA, 20 bp, Artificial Sequence
  LST1 Forward Primer Sequence
ctggccagtttggagtctgt

SEQ ID NO: 160 - DNA, 20 bp, Artificial Sequence
  LST1 Reverse primer Sequence
tccttgctcttttaggcgaa

SEQ ID NO: 161 - DNA, 18 bp, Artificial Sequence
  LTBP2 Forward Primer Sequence
accttggccagagcacag

SEQ ID NO: 162 - DNA, 17 bp, Artificial Sequence
  LTBP2 Reverse primer Sequence
tgggaagggtgggtctg

SEQ ID NO: 163 - DNA, 20 bp, Artificial Sequence
  LYN Forward Primer Sequence
ctgaactcaagtcaccgtgg

SEQ ID NO: 164 - DNA, 20 bp, Artificial Sequence
  LYN Reverse primer Sequence
tccatcgtcactcaagctgt

SEQ ID NO: 165 - DNA, 20 bp, Artificial Sequence
  MAFB Forward Primer Sequence
catagagaacgtggcagcaa

SEQ ID NO: 166 - DNA, 20 bp, Artificial Sequence
  MAFB Reverse primer Sequence
atgcccggaactttttcttt

SEQ ID NO: 167 - DNA, 19 bp, Artificial Sequence
  MMP19 Forward Primer Sequence
gcctcgttgtggcctagag

SEQ ID NO: 168 - DNA, 21 bp, Artificial Sequence
  MMP19 Reverse primer Sequence
atgcggaaagtcaggtgcttc

SEQ ID NO: 169 - DNA, 20 bp, Artificial Sequence
  MMP2 Forward Primer Sequence
cagatgcctggaatgccatc

SEQ ID NO: 170 - DNA, 20 bp, Artificial Sequence
  MMP2 Reverse primer Sequence
gcagcctagccagtcggatt

SEQ ID NO: 171 - DNA, 22 bp, Artificial Sequence
  NEK6 Forward Primer Sequence
caggactgtgtcaaggagatcg

SEQ ID NO: 172 - DNA, 21 bp, Artificial Sequence
  NEK6 Reverse primer Sequence
atgttcagctcgttgtcttcg

SEQ ID NO: 173 - DNA, 21 bp, Artificial Sequence
  NFKBIZ Forward Primer Sequence
acacccacaaaccaactctgg

SEQ ID NO: 174 - DNA, 22 bp, Artificial Sequence
  NFKBIZ Reverse primer Sequence
ggcaaaactgtgattctggacc

SEQ ID NO: 175 - DNA, 20 bp, Artificial Sequence
  NINJ1 Forward Primer Sequence
accgaggagtacgagctcaa

SEQ ID NO: 176 - DNA, 20 bp, Artificial Sequence
  NINJ1 Reverse primer Sequence
gctcttcttgctggcgtaat

SEQ ID NO: 177 - DNA, 20 bp, Artificial Sequence
  NPC2 Forward Primer Sequence
agctacattcctgctcctgg

SEQ ID NO: 178 - DNA, 20 bp, Artificial Sequence
  NPC2 Reverse primer Sequence
tgggctcacattcacttcct

SEQ ID NO: 179 - DNA, 19 bp, Artificial Sequence
  NR4A2 Forward Primer Sequence
cgacatttctgccttctcc

SEQ ID NO: 180 - DNA, 20 bp, Artificial Sequence
  NR4A2 Reverse primer Sequence
ggtaaagtgtccaggaaaag

SEQ ID NO: 181 - DNA, 17 bp, Artificial Sequence
  ODC1 Forward Primer Sequence
ggctgcgactcaggctc

SEQ ID NO: 182 - DNA, 19 bp, Artificial Sequence
  ODC1 Reverse primer Sequence
cccttggaacagcagtgac

SEQ ID NO: 183 - DNA, 20 bp, Artificial Sequence
  OLFML2B Forward Primer Sequence
ccccgaagaagaagatgaca

SEQ ID NO: 184 - DNA, 21 bp, Artificial Sequence
  OLFML2B Reverse primer Sequence
ccatatgtgttctgggtggtc

SEQ ID NO: 185 - DNA, 20 bp, Artificial Sequence
  PDGFA Forward Primer Sequence
tccacgccactaagcatgtg

SEQ ID NO: 186 - DNA, 22 bp, Artificial Sequence
  PDGFA Reverse primer Sequence
cgtaaatgaccgtcctggtctt

SEQ ID NO: 187 - DNA, 20 bp, Artificial Sequence
  PHLDA1 Forward Primer Sequence
ctccaactctgcctgaaagg

SEQ ID NO: 188 - DNA, 22 bp, Artificial Sequence
  PHLDA1 Reverse primer Sequence
tgttttgcttttgatccaagtg

SEQ ID NO: 189 - DNA, 22 bp, Artificial Sequence
  PIM3 Forward Primer Sequence
aaggacgaaaatctgcttgtgg

SEQ ID NO: 190 - DNA, 20 bp, Artificial Sequence
  PIM3 Reverse primer Sequence
cgaagtcggtgtagaccgtg

SEQ ID NO: 191 - DNA, 22 bp, Artificial Sequence
  PLAU Forward Primer Sequence
gggaatggtcacttttaccgag

SEQ ID NO: 192 - DNA, 19 bp, Artificial Sequence
  PLAU Reverse primer Sequence
gggcatggtacgtttgctg

SEQ ID NO: 193 - DNA, 20 bp, Artificial Sequence
  PLAUR Forward Primer Sequence
agccttaccgaggttgtgtg

SEQ ID NO: 194 - DNA, 20 bp, Artificial Sequence
  PLAUR Reverse primer Sequence
aaatgcattcgaggtaacgg

SEQ ID NO: 195 - DNA, 20 bp, Artificial Sequence
  PLD3 Forward Primer Sequence
ggagatctgcctcaatggaa

SEQ ID NO: 196 - DNA, 21 bp, Artificial Sequence
  PLD3 Reverse primer Sequence
ccacgttgagtagagccttca

SEQ ID NO: 197 - DNA, 20 bp, Artificial Sequence
  PMP22 Forward Primer Sequence
tcaggaaatgtccaccactg

SEQ ID NO: 198 - DNA, 20 bp, Artificial Sequence
  PMP22 Reverse primer Sequence
gctgaagatgatcgacagga

SEQ ID NO: 199 - DNA, 20 bp, Artificial Sequence
  PPIB Forward Primer Sequence
aaggacttcatgatccaggg

SEQ ID NO: 200 - DNA, 20 bp, Artificial Sequence
  PPIB Reverse primer Sequence
tgaagttctcatcggggaag

SEQ ID NO: 201 - DNA, 20 bp, Artificial Sequence
  PPIF Forward Primer Sequence
acagggtgatcccttccttc

SEQ ID NO: 202 - DNA, 20 bp, Artificial Sequence
  PPIF Reverse primer Sequence
aagttctcgtcaggaaagcg

SEQ ID NO: 203 - DNA, 21 bp, Artificial Sequence
  PRNP Forward Primer Sequence
cacgactgcgtcaatatcaca

SEQ ID NO: 204 - DNA, 22 bp, Artificial Sequence
  PRNP Reverse primer Sequence
ctccatcatcttaacgtcggtc

SEQ ID NO: 205 - DNA, 21 bp, Artificial Sequence
  RCC2 Forward Primer Sequence
aaggagcgcgtcaaacttgaa

SEQ ID NO: 206 - DNA, 22 bp, Artificial Sequence
  RCC2 Reverse primer Sequence
gcttgctgtttaggcacttctt

SEQ ID NO: 207 - DNA, 21 bp, Artificial Sequence
  REL Forward Primer Sequence
gcagaggggaatgcgttttag

SEQ ID NO: 208 - DNA, 22 bp, Artificial Sequence
  REL Reverse primer Sequence
agaagggtatgttcggttgttg

SEQ ID NO: 209 - DNA, 20 bp, Artificial Sequence
  RGS1 Forward Primer Sequence
ggaaaaacttcttgccaacc

SEQ ID NO: 210 - DNA, 20 bp, Artificial Sequence
  RGS1 Reverse Primer Sequence
tagtcttcacaagccagcca

SEQ ID NO: 211 - DNA, 20 bp, Artificial Sequence
  RHOG Forward Primer Sequence
acgatgcagagcatcaagtg

SEQ ID NO: 212 - DNA, 20 bp, Artificial Sequence
  RHOG Reverse primer Sequence
tttggggaaagcgttagttg

SEQ ID NO: 213 - DNA, 23 bp, Artificial Sequence
  RILPL2 Forward Primer Sequence
acgtgtatgacatctcctacctg

SEQ ID NO: 214 - DNA, 20 bp, Artificial Sequence
  RILPL2 Reverse primer Sequence
acgcggacgactttgaactg

SEQ ID NO: 215 - DNA, 20 bp, Artificial Sequence
  RUNX1 Forward Primer Sequence
tccacaaacccaccgcaagt

SEQ ID NO: 216 - DNA, 19 bp, Artificial Sequence
  RUNX1 Reverse primer Sequence
cgctcggaaaaggacaagc

SEQ ID NO: 217 - DNA, 22 bp, Artificial Sequence
  RUNX2 Forward Primer Sequence
accatggtggagatcatcgccg

SEQ ID NO: 218 - DNA, 24 bp, Artificial Sequence
  RUNX2 Reverse primer Sequence
tcccatctggtacctctccgaggg

SEQ ID NO: 219 - DNA, 22 bp, Artificial Sequence
  Runx3 Forward Primer Sequence
aggcaatgacgagaactactcc

SEQ ID NO: 220 - DNA, 20 bp, Artificial Sequence
  Runx3 Reverse primer Sequence
gtggggttggtgaacacagt

SEQ ID NO: 221 - DNA, 20 bp, Artificial Sequence
  SAMSN1 Forward Primer Sequence
tgctcaagagaaagccatcc

SEQ ID NO: 222 - DNA, 21 bp, Artificial Sequence
  SAMSN1 Reverse primer Sequence
ttattccgaaaacgatcgaaa

SEQ ID NO: 223 - DNA, 23 bp, Artificial Sequence
  SCD Forward Primer Sequence
ttcctacctgcaagttctacacc

SEQ ID NO: 224 - DNA, 20 bp, Artificial Sequence
  SCD Reverse primer Sequence
ccgagctttgtaagagcggt

SEQ ID NO: 225 - DNA, 19 bp, Artificial Sequence
  SDC4 Forward Primer Sequence
tccccaccgaacccaagaa

SEQ ID NO: 226 - DNA, 21 bp, Artificial Sequence
  SDC4 Reverse primer Sequence
ccttgttggacacatcctcac

SEQ ID NO: 227 - DNA, 18 bp, Artificial Sequence
  SH2B3 Forward Primer Sequence
ctggagctcttcgaccca

SEQ ID NO: 228 - DNA, 20 bp, Artificial Sequence
  SH2B3 Reverse primer Sequence
gttgtcaggcatctcaagcc

SEQ ID NO: 229 - DNA, 20 bp, Artificial Sequence
  SMS Forward Primer Sequence
cctcactatggcagcagcac

SEQ ID NO: 230 - DNA, 20 bp, Artificial Sequence
  SMS Reverse primer Sequence
tcctggaaaatggactggag

SEQ ID NO: 231 - DNA, 20 bp, Artificial Sequence
  THBS1 Forward Primer Sequence
caatgccacagttcctgatg

SEQ ID NO: 232 - DNA, 21 bp, Artificial Sequence
  THBS1 Reverse primer Sequence
cacagctcgtagaacaggagg

SEQ ID NO: 233 - DNA, 20 bp, Artificial Sequence
  THY1 Forward Primer Sequence
tcaggaaatggcttttccca

SEQ ID NO: 234 - DNA, 23 bp, Artificial Sequence
  THY1 Reverse primer Sequence
tcctcaatgagatgccataagct

SEQ ID NO: 235 - DNA, 20 bp, Artificial Sequence
  TNFAIP2 Forward Primer Sequence
cacctacatgctgctgctct

SEQ ID NO: 236 - DNA, 19 bp, Artificial Sequence
  TNFAIP2 Reverse primer Sequence
cccataccctgcagctcac

SEQ ID NO: 237 - DNA, 21 bp, Artificial Sequence
  TNFAIP3 Forward Primer Sequence
ttgtcctcagtttcgggagat

SEQ ID NO: 238 - DNA, 22 bp, Artificial Sequence
  TNFAIP3 Reverse primer Sequence
acttctcgacaccagttgagtt

SEQ ID NO: 239 - DNA, 21 bp, Artificial Sequence
  TTYH2 Forward Primer Sequence
cccctgtctccgagtacatga

SEQ ID NO: 240 - DNA, 21 bp, Artificial Sequence
  TTYH2 Reverse primer Sequence
ctcccgattagtggcacgttc

SEQ ID NO: 241 - DNA, 23 bp, Artificial Sequence
  UNC93B1 Forward Primer Sequence
ttttggaacgaagtggatgatgt

SEQ ID NO: 242 - DNA, 19 bp, Artificial Sequence
  UNC93B1 Reverse primer Sequence
ggcacaagcgtgtagtagc

SEQ ID NO: 243 - DNA, 20 bp, Artificial Sequence
  VAMP8 Forward Primer Sequence
acttggaacatctccgcaac

SEQ ID NO: 244 - DNA, 20 bp, Artificial Sequence
  VAMP8 Reverse primer Sequence
cttccaccagaatttccgag

SEQ ID NO: 245 - DNA, 19 bp, Artificial Sequence
  ZSWIM6 Forward Primer Sequence
aagcggctgcgtagacaac

SEQ ID NO: 246 - DNA, 21 bp, Artificial Sequence
  ZSWIM6 Reverse primer Sequence
ggctccgattgtattgcaggt

SEQ ID NO: 247 - RNA, 25 nt, Artificial Sequence
  RUNX1 siRNA sequence
ccuuucauguuaaucaaacaaguga

SEQ ID NO: 248 - RNA, 27 nt, Artificial Sequence
  RUNX1 siRNA sequence
ucacuuguuugauuaacaugaaaggga

SEQ ID NO: 249 - RNA, 25 nt, Artificial Sequence
  RUNX1 siRNA sequence
acuagaugaucagaccaagcccggg

SEQ ID NO: 250 - RNA, 27 nt, Artificial Sequence
  RUNX1 siRNA sequence
cccgggcuuggucugaucaucuaguuu

SEQ ID NO: 251 - DNA, 24 bp, Artificial Sequence
  PIM3 siRNA sequence
ccugagcguuuaauuuauucagta

SEQ ID NO: 252 - RNA, 27 nt, Artificial Sequence
  PIM3 siRNA sequence
uacugaauaaauuaaacgcucaggcuc

SEQ ID NO: 253 - DNA, 25 bp, Artificial Sequence
  PIM3 siRNA sequence
ggcgugcuucucuacgauauggugt

SEQ ID NO: 254 - RNA, 27 nt, Artificial Sequence
  PIM3 siRNA sequence
acaccauaucguagagaagcacgccca

SEQ ID NO: 255 - DNA, 23 bp, Artificial Sequence
  RUNX1 guide RNA
gatgagcgaggcgttgccgctgg

SEQ ID NO: 256 - DNA, 23 bp, Artificial Sequence
  RUNX1 guide RNA
tagatgatcagaccaagcccggg

SEQ ID NO: 257 - DNA, 23 bp, Artificial Sequence
  RUNX1 guide RNA
tggcaatgatgaaaactactcgg